European Patent Specification EP 3 911 354 B1, published July 19, 2023. Title: AAV-MEDIATED GENE THERAPY RESTORING THE OTOFERLIN GENE. Applicant: INSTITUT PASTEUR. The sequence listing filed with the application follows.

SEQUENCE LISTING (24 sequences)

SEQ ID NO: 1 - protein, 1997 aa, homo sapiens
MALLIHLKTVSELRGRGDRIAKVTFRGQSFYSRVLENCEDVADFDETFRWPVASSIDRNEMLEIQVFNYSKVFSNKLIGTFRMVLQKVVEESHVEVTDTLIDDNNAIIKTSLCVEVRYQATDGTVGSWDDGDFLGDESLQEEEKDSQETDGLLPGSRPSSRPPGEKSFRRAGRSVFSAMKLGKNRSHKEEPQRPDEPAVLEMEDLDHLAIRLGDGLDPDSVSLASVTALTTNVSNKRSKPDIKMEPSAGRPMDYQVSITVIEARQLVGLNMDPVVCVEVGDDKKYTSMKESTNCPYYNEYFVFDFHVSPDVMFDKIIKISVIHSKNLLRSGTLVGSFKMDVGTVYSQPEHQFHHKWAILSDPDDISSGLKGYVKCDVAVVGKGDNIKTPHKANETDEDDIEGNLLLPEGVPPERQWARFYVKIYRAEGLPRMNTSLMANVKKAFIGENKDLVDPYVQVFFAGQKGKTSVQKSSYEPLWNEQVVFTDLFPPLCKRMKVQIRDSDKVNDVAIGTHFIDLRKISNDGDKGFLPTLGPAWVNMYGSTRNYTLLDEHQDLNEGLGEGVSFRARLLLGLAVEIVDTSNPELTSSTEVQVEQATPISESCAGKMEEFFLFGAFLEASMIDRRNGDKPITFEVTIGNYGNEVDGLSRPQRPRPRKEPGDEEEVDLIQNASDDEAGDAGDLASVSSTPPMRPQVTDRNYFHLPYLERKPCIYIKSWWPDQRRRLYNANIMDHIADKLEEGLNDIQEMIKTEKSYPERRLRGVLEELSCGCCRFLSLADKDQGHSSRTRLDRERLKSCMRELENMGQQARMLRAQVKRHTVRDKLRLCQNFLQKLRFLADEPQHSIPDIFIWMMSNNKRVAYARVPSKDLLFSIVEEETGKDCAKVKTLFLKLPGKRGFGSAGWTVQAKVELYLWLGLSKQRKEFLCGLPCGFQEVKAAQGLGLHAFPPVSLVYTKKQAFQLRAHMYQARSLFAADSSGLSDPFARVFFINQSQCTEVLNETLCPTWDQMLVFDNLELYGEAHELRDDPPIIVIEIYDQDSMGKADFMGRTFAKPLVKMADEAYCPPRFPPQLEYYQIYRGNATAGDLLAAFELLQIGPAGKADLPPINGPVDVDRGPIMPVPMGIRPVLSKYRVEVLFWGLRDLKRVNLAQVDRPRVDIECAGKGVQSSLIHNYKKNPNFNTLVKWFEVDLPENELLHPPLNIRVVDCRAFGRYTLVGSHAVSSLRRFIYRPPDRSAPSWNTTVRLLRRCRVLCNGGSSSHSTGEVVVTMEPEVPIKKLETMVKLDATSEAVVKVDVAEEEKEKKKKKKGTAEEPEEEEPDESMLDWWSKYFASIDTMKEQLRQQEPSGIDLEEKEEVDNTEGLKGSMKGKEKARAAKEEKKKKTQSSGSGQGSEAPEKKKPKIDELKVYPKELESEFDNFEDWLHTFNLLRGKTGDDEDGSTEEERIVGRFKGSLCVYKVPLPEDVSREAGYDSTYGMFQGIPSNDPINVLVRVYVVRATDLHPADINGKADPYIAIRLGKTDIRDKENYISKQLNPVFGKSFDIEASFPMESMLTVAVYDWDLVGTDDLIGETKIDLENRFYSKHRATCGIAQTYSTHGYNIWRDPMKPSQILTRLCKDGKVDGPHFGPPGRVKVANRVFTGPSEIEDENGQRKPTDEHVALLALRHWEDIPRAGCRLVPEHVETRPLLNPDKPGIEQGRLELWVDMFPMDMPAPGTPLDISPRKPKKYELRVIIWNTDEVVLEDDDFFTGEKSSDIFVRGWLKGQQEDKQDTDVHYHSLTGEGNFNWRYLFPFDYLAAEEKIVISKKESMFSWDETEYKIPARLTLQIWDADHFSADDFLGAIELDLNRFPRGAKTAKQCTMEMATGEVDVPLVSIFKQKRVKGWWPLLARNENDEFELTGKVEAELHLLTAEEAEKNPVGLARNEPDPLEKPNRPDTSFIWFLNPLKSARYFLWHTYRWLLLKLLLLLLLLLLLALFLYSVPGYLVKKILGA

SEQ ID NO: 2 - DNA, 7171 bp, homo sapiens
atcggaggggggtcgggaggaggaggaggaggcagcggcagagaagagagaggcgtgtgagccgtgctccaccggctagctccttcccgctgctcctgcctggcagtgccaggcagcccacaccagcatggccttgctcatccacctcaagacagtctcggagctgcggggcaggggcgaccggatcgccaaagtgactttccgagggcaatccttctactctcgggtcctggagaactgtgaggatgtggctgactttgatgagacatttcggtggccggtggccagcagcatcgacagaaatgagatgctggagattcaggttttcaactacagcaaagtcttcagcaacaagctcatcgggaccttccgcatggtgctgcagaaggtggtagaggagagccatgtggaggtgactgacacgctgattgatgacaacaatgctatcatcaagaccagcctgtgcgtggaggtccggtatcaggccactgacggcacagtgggctcctgggacgatggggacttcctgggagatgagtctcttcaagaggaagagaaggacagccaagagacggatggactgctcccaggctcccggcccagctcccggcccccaggagagaagagcttccggagagccgggaggagcgtgttctccgccatgaagctcggcaaaaaccggtctcacaaggaggagccccaaagaccagatgaaccggcggtgctggagatggaagaccttgaccatctggccattcggctaggagatggactggatcccgactcggtgtctctagcctcagtcacagctctcaccactaatgtctccaacaagcgatctaagccagacattaagatggagccaagtgctgggcggcccatggattaccaggtcagcatcacggtgatcgaggcccggcagctggtgggcttgaacatggaccctgtggtgtgcgtggaggtgggtgacgacaagaagtacacatccatgaaggagtccactaactgcccctattacaacgagtacttcgtcttcgacttccatgtctctccggatgtcatgtttgacaagatcatcaagatttcggtgattcactccaagaacctgctgcgcagtggcaccctggtgggctccttcaaaatggacgtgggaaccgtgtactcgcagccagagcaccagttccatcacaagtgggccatcctgtctgaccccgatgacatctcctcggggctgaagggctacgtgaagtgtgacgttgccgtggtgggcaaaggggacaacatcaagacgccccacaaggccaatgagaccgacgaagatgacattgaggggaacttgctgctccccgagggggtgccccccgaacgccagtgggcccggttctatgtgaaaatttaccgagcagaggggctgccccgtatgaacacaagcctcatggccaatgtaaagaaggctttcatcggtgaaaacaaggacctcgtggacccctacgtgcaagtcttctttgctggccagaagggcaagacttcagtgcagaagagcagctatgagcccctgtggaatgagcaggtcgtctttacagacctcttccccccactctgcaaacgcatgaaggtgcagatccgagactcggacaaggtcaacgacgtggccatcggcacccacttcattgacctgcgcaagatttctaatgacggagacaaaggcttcctgcccacactgggcccagcctgggtgaacatgtacggctccacacgtaactacacgctgctggatgagcatcaggacctgaacgagggcctgggggagggtgtgtccttccgggcccggctcctgctgggcctggctgtggagatcgtagacacctccaaccctgagctcaccagctccacagaggtgcaggtggagcaggccacgcccatctcggagagctgtgcaggtaaaatggaagaattctttctctttggagccttcctggaggcctcaatgatcgaccggagaaacggagacaagcccatcacctttgaggtcaccataggcaactatgggaacgaagttgatggcctgtcccggccccagcggcctcggccccggaaggagccgggggatgaggaagaagtagacctgattcagaacgcaagtgatgacgaggccggtgatgccggggacctggcctcagtctcctccactccaccaatgcggccccaggtcaccgacaggaactacttccatctgccctacctggagcgaaagccctgcatctacatcaagagctggtggccggaccagcgccgccgcctctacaatgccaacatcatggaccacattgccgacaagctggaagaaggcctgaacgacatacaggagatgatcaaaacggagaagtcctaccctgagcgtcgcctgcggggcgtcctggaggagctgagctgtggctgctgccgcttcctctccctcgctgacaaggaccagggccactcatcccgcaccaggcttgaccgggagcgcctcaagtcctgcatgagggagctggaaaacatggggcagcaggccaggatgctgcgggcccaggtgaagcggcacacggtgcgggacaagctgaggctgtgccagaacttcctgcagaagctgcgcttcctggcggacgagccccagcacagcattcccgacatcttcatctggatgatgagcaacaacaagcgtgtcgcctatgcccgtgtgccctccaaggacctgctcttctccatcgtggaggaggagactggcaaggactgcgccaaggtcaagacgctcttccttaagctgccagggaagcggggcttcggctcggcaggctggacagtgcaggccaaggtggagctgtacctgtggctgggcctcagcaaacagcgcaaggagttcctgtgcggcctgccctgtggcttccaggaggtcaaggcagcccagggcctgggcctgcatgccttcccacccgtcagcctggtctacaccaagaagcaggcgttccagctccgagcgcacatgtaccaggcccgcagcctctttgccgccgacagcagcggactctcagacccctttgcccgcgtcttcttcatcaatcagagtcagtgcacagaggtgctgaatgagaccctgtgtcccacctgggaccagatgctggtgttcgacaacctggagctctatggtgaagctcatgagctgagggacgatccgcccatcattgtcattgaaatctatgaccaggattccatgggcaaagctgacttcatgggccggaccttcgccaaacccctggtgaagatggcagacgaggcgtactgcccaccccgcttcccacctcagctcgagtactaccagatctaccgtggcaacgccacagctggagacctgctggcggccttcgagctgctgcagattggaccagcagggaaggctgacctgccccccatcaatggcccggtggacgtggaccgaggtcccatcatgcccgtgcccatgggcatccggcccgtgctcagcaagtaccgagtggaggtgctgttctggggcctacgggacctaaagcgggtgaacctggcccaggtggaccggccacgggtggacatcgagtgtgcagggaagggggtgcagtcgtccctgatccacaattataagaagaaccccaacttcaacaccctcgtcaagtggtttgaagtggacctcccagagaacgagctgctgcacccgcccttgaacatccgtgtggtggactgccgggccttcggtcgctacacactggtgggctcccatgccgtcagctccctgcgacgcttcatctaccggcccccagaccgctcggcccccagctggaacaccacggtcaggcttctccggcgctgccgtgtgctgtgcaatgggggctcctcctctcactccacaggggaggttgtggtgactatggagccagaggtacccatcaagaaactggagaccatggtgaagctggacgcgacttctgaagctgttgtcaaggtggatgtggctgaggaggagaaggagaagaagaagaagaagaagggcactgcggaggagccagaggaggaggagccagacgagagcatgctggactggtggtccaagtactttgcctccattgacaccatgaaggagcaacttcgacaacaagagccctctggaattgacttggaggagaaggaggaagtggacaataccgagggcctgaaggggtcaatgaagggcaaggagaaggcaagggctgccaaagaggagaagaagaagaaaactcagagctctggctctggccaggggtccgaggcccccgagaagaagaaacccaagattgatgagcttaaggtataccccaaagagctggagtccgagtttgataactttgaggactggctgcacactttcaacttgcttcggggcaagaccggggatgatgaggatggctccaccgaggaggagcgcattgtgggacgcttcaagggctccctctgcgtgtacaaagtgccactcccagaggacgtgtcccgggaagccggctacgactccacctacggcatgttccagggcatcccgagcaatgaccccatcaatgtgctggtccgagtctatgtggtccgggccacggacctgcaccctgctgacatcaacggcaaagctgacccctacatcgccatccggctaggcaagactgacatccgcgacaaggagaactacatctccaagcagctcaaccctgtctttgggaagtcctttgacatcgaggcctccttccccatggaatccatgctgacggtggctgtgtatgactgggacctggtgggcactgatgacctcattggggaaaccaagatcgacctggagaaccgcttctacagcaagcaccgcgccacctgcggcatcgcccagacctactccacacatggctacaatatctggcgggaccccatgaagcccagccagatcctgacccgcctctgcaaagacggcaaagtggacggcccccactttgggccccctgggagagtgaaggtggccaaccgcgtcttcactgggccctctgagattgaggacgagaacggtcagaggaagcccacagacgagcatgtggcgctgttggccctgaggcactgggaggacatcccccgcgcaggctgccgcctggtgccagagcatgtggagacgaggccgctgctcaaccccgacaagccgggcatcgagcagggccgcctggagctgtgggtggacatgttccccatggacatgccagcccctgggacgcctctggacatctcacctcggaagcccaagaagtacgagctgcgggtcatcatctggaacacagatgaggtggtcttggaggacgacgacttcttcacaggggagaagtccagtgacatcttcgtgagggggtggctgaagggccagcaggaggacaagcaggacacagacgtccactaccactccctcactggcgagggcaacttcaactggcgctacctgttccccttcgactacctggcggcggaggagaagatcgtcatctccaagaaggagtccatgttctcctgggacgagaccgagtacaagatccccgcgcggctcaccctgcagatctgggatgcggaccacttctccgctgacgacttcctgggggccatcgagctggacctgaaccggttcccgcggggcgcaaagacagccaagcagtgcaccatggagatggccaccggggaggtggacgtgcccctcgtgtccatcttcaagcaaaagcgcgtcaaaggctggtggcccctcctggcccgcaatgagaacgatgagtttgagctcacgggcaaggtggaggctgagctgcatttactgacagcagaggaggcagagaagaacccagtgggcctggcccgcaatgaacctgaccccctagagaaacccaaccggcccgacacgagcttcatctggttcctgaaccctctcaagtcggctcgctacttcttgtggcacacgtatcgctggctgctcctcaaactgttgctgctcctgctgctgctcctcctcctcgccctgttcctctactctgtgcctggctacctggtcaagaaaatcctcggggcctgagcccagtggcctcctggccggcccgacacggccttcgtctggttcctcaaccctctcaagtccatcaagtacctcatctgcacccggtacaagtggctcatcatcaagatcgtgctggcgctgttggggctgctcatgttggggctcttcctctacagcctccctggctacatggtcaaaaagctccttggggcatgaaggccgccagctcccgccagccgctccccagccctgccgcatttcctttcagtggcttggactctttcccatctcccctggggagcctgaggagcccagcgtccactcttcatgccttgggccgagcctgcctcctgcttgcgggggccgcctgtcctcactgccccaggctgcggcttgcccagtcccgcccctctgacccctgcctgtgggctggggagccttggatggggtggggacctggaatgggtctctcttgccccacctggctgaggcgccacccttcttcaggcccaggctccagaggaagactcctgaaaccctccccaggtcttccaagtacaggattgaagctttagtgaaattaaccaaggaccatgggtcagtgcccagggctttaaaaagaatgaacgagcaaaaggtatccccgccgtgacccctgcagatagcaccggtctttgatccgcagcaggggccagaccctgcccacaagtcccagcgcggctgcttctgccactgctgggctccacttggctcctctcacttcccagggggtcgcctgtcctgcctgtgggtttccatggcttcccagagctccctctgccccagccagcgcctccaggcccagctgaggagctgtgagaagcagcagaggggactccccatcccgggcacaccctgtcctcccacccctgcccccttgcccttccagccctttcagctgcagctgggagctggcccgtcaagtgctgcccctgcctgtgtctgggtttctgttggctgtttttcttttcttgagtggtgatttttctctaaataaaagaagtcaagcactgaaaaaaaaaaaaaaaa

SEQ ID NO: 3 - DNA, 2676 bp, homo sapiens
atggccttgctcatccacctcaagacagtctcggagctgcggggcaggggcgaccggatcgccaaagtgactttccgagggcaatccttctactctcgggtcctggagaactgtgaggatgtggctgactttgatgagacatttcggtggccggtggccagcagcatcgacagaaatgagatgctggagattcaggttttcaactacagcaaagtcttcagcaacaagctcatcgggaccttccgcatggtgctgcagaaggtggtagaggagagccatgtggaggtgactgacacgctgattgatgacaacaatgctatcatcaagaccagcctgtgcgtggaggtccggtatcaggccactgacggcacagtgggctcctgggacgatggggacttcctgggagatgagtctcttcaagaggaagagaaggacagccaagagacggatggactgctcccaggctcccggcccagctcccggcccccaggagagaagagcttccggagagccgggaggagcgtgttctccgccatgaagctcggcaaaaaccggtctcacaaggaggagccccaaagaccagatgaaccggcggtgctggagatggaagaccttgaccatctggccattcggctaggagatggactggatcccgactcggtgtctctagcctcagtcacagctctcaccactaatgtctccaacaagcgatctaagccagacattaagatggagccaagtgctgggcggcccatggattaccaggtcagcatcacggtgatcgaggcccggcagctggtgggcttgaacatggaccctgtggtgtgcgtggaggtgggtgacgacaagaagtacacatccatgaaggagtccactaactgcccctattacaacgagtacttcgtcttcgacttccatgtctctccggatgtcatgtttgacaagatcatcaagatttcggtgattcactccaagaacctgctgcgcagtggcaccctggtgggctccttcaaaatggacgtgggaaccgtgtactcgcagccagagcaccagttccatcacaagtgggccatcctgtctgaccccgatgacatctcctcggggctgaagggctacgtgaagtgtgacgttgccgtggtgggcaaaggggacaacatcaagacgccccacaaggccaatgagaccgacgaagatgacattgaggggaacttgctgctccccgagggggtgccccccgaacgccagtgggcccggttctatgtgaaaatttaccgagcagaggggctgccccgtatgaacacaagcctcatggccaatgtaaagaaggctttcatcggtgaaaacaaggacctcgtggacccctacgtgcaagtcttctttgctggccagaagggcaagacttcagtgcagaagagcagctatgagcccctgtggaatgagcaggtcgtctttacagacctcttccccccactctgcaaacgcatgaaggtgcagatccgagactcggacaaggtcaacgacgtggccatcggcacccacttcattgacctgcgcaagatttctaatgacggagacaaaggcttcctgcccacactgggcccagcctgggtgaacatgtacggctccacacgtaactacacgctgctggatgagcatcaggacctgaacgagggcctgggggagggtgtgtccttccgggcccggctcctgctgggcctggctgtggagatcgtagacacctccaaccctgagctcaccagctccacagaggtgcaggtggagcaggccacgcccatctcggagagctgtgcaggtaaaatggaagaattctttctctttggagccttcctggaggcctcaatgatcgaccggagaaacggagacaagcccatcacctttgaggtcaccataggcaactatgggaacgaagttgatggcctgtcccggccccagcggcctcggccccggaaggagccgggggatgaggaagaagtagacctgattcagaacgcaagtgatgacgaggccggtgatgccggggacctggcctcagtctcctccactccaccaatgcggccccaggtcaccgacaggaactacttccatctgccctacctggagcgaaagccctgcatctacatcaagagctggtggccggaccagcgccgccgcctctacaatgccaacatcatggaccacattgccgacaagctggaagaaggcctgaacgacatacaggagatgatcaaaacggagaagtcctaccctgagcgtcgcctgcggggcgtcctggaggagctgagctgtggctgctgccgcttcctctccctcgctgacaaggaccagggccactcatcccgcaccaggcttgaccgggagcgcctcaagtcctgcatgagggagctggaaaacatggggcagcaggccaggatgctgcgggcccaggtgaagcggcacacggtgcgggacaagctgaggctgtgccagaacttcctgcagaagctgcgcttcctggcggacgagccccagcacagcattcccgacatcttcatctggatgatgagcaacaacaagcgtgtcgcctatgcccgtgtgccctccaaggacctgctcttctccatcgtggaggaggagactggcaaggactgcgccaaggtcaagacgctcttccttaag

SEQ ID NO: 4 - DNA, 3318 bp, homo sapiens
ctgccagggaagcggggcttcggctcggcaggctggacagtgcaggccaaggtggagctgtacctgtggctgggcctcagcaaacagcgcaaggagttcctgtgcggcctgccctgtggcttccaggaggtcaaggcagcccagggcctgggcctgcatgccttcccacccgtcagcctggtctacaccaagaagcaggcgttccagctccgagcgcacatgtaccaggcccgcagcctctttgccgccgacagcagcggactctcagacccctttgcccgcgtcttcttcatcaatcagagtcagtgcacagaggtgctgaatgagaccctgtgtcccacctgggaccagatgctggtgttcgacaacctggagctctatggtgaagctcatgagctgagggacgatccgcccatcattgtcattgaaatctatgaccaggattccatgggcaaagctgacttcatgggccggaccttcgccaaacccctggtgaagatggcagacgaggcgtactgcccaccccgcttcccacctcagctcgagtactaccagatctaccgtggcaacgccacagctggagacctgctggcggccttcgagctgctgcagattggaccagcagggaaggctgacctgccccccatcaatggcccggtggacgtggaccgaggtcccatcatgcccgtgcccatgggcatccggcccgtgctcagcaagtaccgagtggaggtgctgttctggggcctacgggacctaaagcgggtgaacctggcccaggtggaccggccacgggtggacatcgagtgtgcagggaagggggtgcagtcgtccctgatccacaattataagaagaaccccaacttcaacaccctcgtcaagtggtttgaagtggacctcccagagaacgagctgctgcacccgcccttgaacatccgtgtggtggactgccgggccttcggtcgctacacactggtgggctcccatgccgtcagctccctgcgacgcttcatctaccggcccccagaccgctcggcccccagctggaacaccacggtcaggcttctccggcgctgccgtgtgctgtgcaatgggggctcctcctctcactccacaggggaggttgtggtgactatggagccagaggtacccatcaagaaactggagaccatggtgaagctggacgcgacttctgaagctgttgtcaaggtggatgtggctgaggaggagaaggagaagaagaagaagaagaagggcactgcggaggagccagaggaggaggagccagacgagagcatgctggactggtggtccaagtactttgcctccattgacaccatgaaggagcaacttcgacaacaagagccctctggaattgacttggaggagaaggaggaagtggacaataccgagggcctgaaggggtcaatgaagggcaaggagaaggcaagggctgccaaagaggagaagaagaagaaaactcagagctctggctctggccaggggtccgaggcccccgagaagaagaaacccaagattgatgagcttaaggtataccccaaagagctggagtccgagtttgataactttgaggactggctgcacactttcaacttgcttcggggcaagaccggggatgatgaggatggctccaccgaggaggagcgcattgtgggacgcttcaagggctccctctgcgtgtacaaagtgccactcccagaggacgtgtcccgggaagccggctacgactccacctacggcatgttccagggcatcccgagcaatgaccccatcaatgtgctggtccgagtctatgtggtccgggccacggacctgcaccctgctgacatcaacggcaaagctgacccctacatcgccatccggctaggcaagactgacatccgcgacaaggagaactacatctccaagcagctcaaccctgtctttgggaagtcctttgacatcgaggcctccttccccatggaatccatgctgacggtggctgtgtatgactgggacctggtgggcactgatgacctcattggggaaaccaagatcgacctggagaaccgcttctacagcaagcaccgcgccacctgcggcatcgcccagacctactccacacatggctacaatatctggcgggaccccatgaagcccagccagatcctgacccgcctctgcaaagacggcaaagtggacggcccccactttgggccccctgggagagtgaaggtggccaaccgcgtcttcactgggccctctgagattgaggacgagaacggtcagaggaagcccacagacgagcatgtggcgctgttggccctgaggcactgggaggacatcccccgcgcaggctgccgcctggtgccagagcatgtggagacgaggccgctgctcaaccccgacaagccgggcatcgagcagggccgcctggagctgtgggtggacatgttccccatggacatgccagcccctgggacgcctctggacatctcacctcggaagcccaagaagtacgagctgcgggtcatcatctggaacacagatgaggtggtcttggaggacgacgacttcttcacaggggagaagtccagtgacatcttcgtgagggggtggctgaagggccagcaggaggacaagcaggacacagacgtccactaccactccctcactggcgagggcaacttcaactggcgctacctgttccccttcgactacctggcggcggaggagaagatcgtcatctccaagaaggagtccatgttctcctgggacgagaccgagtacaagatccccgcgcggctcaccctgcagatctgggatgcggaccacttctccgctgacgacttcctgggggccatcgagctggacctgaaccggttcccgcggggcgcaaagacagccaagcagtgcaccatggagatggccaccggggaggtggacgtgcccctcgtgtccatcttcaagcaaaagcgcgtcaaaggctggtggcccctcctggcccgcaatgagaacgatgagtttgagctcacgggcaaggtggaggctgagctgcatttactgacagcagaggaggcagagaagaacccagtgggcctggcccgcaatgaacctgaccccctagagaaacccaaccggcccgacacgagcttcatctggttcctgaaccctctcaagtcggctcgctacttcttgtggcacacgtatcgctggctgctcctcaaactgttgctgctcctgctgctgctcctcctcctcgccctgttcctctactctgtgcctggctacctggtcaagaaaatcctcggggcctga

SEQ ID NO: 5 - protein, 1997 aa, homo sapiens
MALLIHLKTVSELRGRGDRIAKVTFRGQSFYSRVLENCEDVADFDETFRWPVASSIDRNEMLEIQVFNYSKVFSNKLIGTFRMVLQKVVEESHVEVTDTLIDDNNAIIKTSLCVEVRYQATDGTVGSWDDGDFLGDESLQEEEKDSQETDGLLPGSRPSSRPPGEKSFRRAGRSVFSAMKLGKNRSHKEEPQRPDEPAVLEMEDLDHLAIRLGDGLDPDSVSLASVTALTTNVSNKRSKPDIKMEPSAGRPMDYQVSITVIEARQLVGLNMDPVVCVEVGDDKKYTSMKESTNCPYYNEYFVFDFHVSPDVMFDKIIKISVIHSKNLLRSGTLVGSFKMDVGTVYSQPEHQFHHKWAILSDPDDISSGLKGYVKCDVAVVGKGDNIKTPHKANETDEDDIEGNLLLPEGVPPERQWARFYVKIYRAEGLPRMNTSLMANVKKAFIGENKDLVDPYVQVFFAGQKGKTSVQKSSYEPLWNEQVVFTDLFPPLCKRMKVQIRDSDKVNDVAIGTHFIDLRKISNDGDKGFLPTLGPAWVNMYGSTRNYTLLDEHQDLNEGLGEGVSFRARLLLGLAVEIVDTSNPELTSSTEVQVEQATPISESCAGKMEEFFLFGAFLEASMIDRRNGDKPITFEVTIGNYGNEVDGLSRPQRPRPRKEPGDEEEVDLIQNASDDEAGDAGDLASVSSTPPMRPQVTDRNYFHLPYLERKPCIYIKSWWPDQRRRLYNANIMDHIADKLEEGLNDIQEMIKTEKSYPERRLRGVLEELSCGCCRFLSLADKDQGHSSRTRLDRERLKSCMRELENMGQQARMLRAQVKRHTVRDKLRLCQNFLQKLRFLADEPQHSIPDIFIWMMSNNKRVAYARVPSKDLLFSIVEEETGKDCAKVKTLFLKLPGKRGFGSAGWTVQAKVELYLWLGLSKQRKEFLCGLPCGFQEVKAAQGLGLHAFPPVSLVYTKKQAFQLRAHMYQARSLFAADSSGLSDPFARVFFINQSQCTEVLNETLCPTWDQMLVFDNLELYGEAHELRDDPPIIVIEIYDQDSMGKADFMGRTFAKPLVKMADEAYCPPRFPPQLEYYQIYRGNATAGDLLAAFELLQIGPAGKADLPPINGPVDVDRGPIMPVPMGIRPVLSKYRVEVLFWGLRDLKRVNLAQVDRPRVDIECAGKGVQSSLIHNYKKNPNFNTLVKWFEVDLPENELLHPPLNIRVVDCRAFGRYTLVGSHAVSSLRRFIYRPPDRSAPSWNTTVRLLRRCRVLCNGGSSSHSTGEVVVTMEPEVPIKKLETMVKLDATSEAVVKVDVAEEEKEKKKKKKGTAEEPEEEEPDESMLDWWSKYFASIDTMKEQLRQQEPSGIDLEEKEEVDNTEGLKGSMKGKEKARAAKEEKKKKTQSSGSGQGSEAPEKKKPKIDELKVYPKELESEFDNFEDWLHTFNLLRGKTGDDEDGSTEEERIVGRFKGSLCVYKVPLPEDVSREAGYDSTYGMFQGIPSNDPINVLVRVYVVRATDLHPADINGKADPYIAIRLGKTDIRDKENYISKQLNPVFGKSFDIEASFPMESMLTVAVYDWDLVGTDDLIGETKIDLENRFYSKHRATCGIAQTYSTHGYNIWRDPMKPSQILTRLCKDGKVDGPHFGPPGRVKVANRVFTGPSEIEDENGQRKPTDEHVALLALRHWEDIPRAGCRLVPEHVETRPLLNPDKPGIEQGRLELWVDMFPMDMPAPGTPLDISPRKPKKYELRVIIWNTDEVVLEDDDFFTGEKSSDIFVRGWLKGQQEDKQDTDVHYHSLTGEGNFNWRYLFPFDYLAAEEKIVISKKESMFSWDETEYKIPARLTLQIWDADHFSADDFLGAIELDLNRFPRGAKTAKQCTMEMATGEVDVPLVSIFKQKRVKGWWPLLARNENDEFELTGKVEAELHLLTAEEAEKNPVGLARNEPDPLEKPNRPDTAFVWFLNPLKSIKYLICTRYKWLIIKIVLALLGLLMLGLFLYSLPGYMVKKLLGA

SEQ ID NO: 6 - protein, 1230 aa, homo sapiens
MIKTEKSYPERRLRGVLEELSCGCCRFLSLADKDQGHSSRTRLDRERLKSCMRELENMGQQARMLRAQVKRHTVRDKLRLCQNFLQKLRFLADEPQHSIPDIFIWMMSNNKRVAYARVPSKDLLFSIVEEETGKDCAKVKTLFLKLPGKRGFGSAGWTVQAKVELYLWLGLSKQRKEFLCGLPCGFQEVKAAQGLGLHAFPPVSLVYTKKQAFQLRAHMYQARSLFAADSSGLSDPFARVFFINQSQCTEVLNETLCPTWDQMLVFDNLELYGEAHELRDDPPIIVIEIYDQDSMGKADFMGRTFAKPLVKMADEAYCPPRFPPQLEYYQIYRGNATAGDLLAAFELLQIGPAGKADLPPINGPVDVDRGPIMPVPMGIRPVLSKYRVEVLFWGLRDLKRVNLAQVDRPRVDIECAGKGVQSSLIHNYKKNPNFNTLVKWFEVDLPENELLHPPLNIRVVDCRAFGRYTLVGSHAVSSLRRFIYRPPDRSAPSWNTTGEVVVTMEPEVPIKKLETMVKLDATSEAVVKVDVAEEEKEKKKKKKGTAEEPEEEEPDESMLDWWSKYFASIDTMKEQLRQQEPSGIDLEEKEEVDNTEGLKGSMKGKEKARAAKEEKKKKTQSSGSGQGSEAPEKKKPKIDELKVYPKELESEFDNFEDWLHTFNLLRGKTGDDEDGSTEEERIVGRFKGSLCVYKVPLPEDVSREAGYDSTYGMFQGIPSNDPINVLVRVYVVRATDLHPADINGKADPYIAIRLGKTDIRDKENYISKQLNPVFGKSFDIEASFPMESMLTVAVYDWDLVGTDDLIGETKIDLENRFYSKHRATCGIAQTYSTHGYNIWRDPMKPSQILTRLCKDGKVDGPHFGPPGRVKVANRVFTGPSEIEDENGQRKPTDEHVALLALRHWEDIPRAGCRLVPEHVETRPLLNPDKPGIEQGRLELWVDMFPMDMPAPGTPLDISPRKPKKYELRVIIWNTDEVVLEDDDFFTGEKSSDIFVRGWLKGQQEDKQDTDVHYHSLTGEGNFNWRYLFPFDYLAAEEKIVISKKESMFSWDETEYKIPARLTLQIWDADHFSADDFLGAIELDLNRFPRGAKTAKQCTMEMATGEVDVPLVSIFKQKRVKGWWPLLARNENDEFELTGKVEAELHLLTAEEAEKNPVGLARNEPDPLEKPNRPDTSFIWFLNPLKSARYFLWHTYRWLLLKLLLLLLLLLLLALFLYSVPGYLVKKILGA

SEQ ID NO: 7 - protein, 1992 aa, musc musculus
MALIVHLKTVSELRGKGDRIAKVTFRGQSFYSRVLENCEGVADFDETFRWPVASSIDRNEVLEIQIFNYSKVFSNKLIGTFCMVLQKVVEENRVEVTDTLMDDSNAIIKTSLSMEVRYQATDGTVGPWDDGDFLGDESLQEEKDSQETDGLLPGSRPSTRISGEKSFRSKGREKTKGGRDGEHKAGRSVFSAMKLGKTRSHKEEPQRQDEPAVLEMEDLDHLAIQLGDGLDPDSVSLASVTALTSNVSNKRSKPDIKMEPSAGRPMDYQVSITVIEARQLVGLNMDPVVCVEVGDDKKYTSMKESTNCPYYNEYFVFDFHVSPDVMFDKIIKISVIHSKNLLRSGTLVGSFKMDVGTVYSQPEHQFHHKWAILSDPDDISAGLKGYVKCDVAVVGKGDNIKTPHKANETDEDDIEGNLLLPEGVPPERQWARFYVKIYRAEGLPRMNTSLMANVKKAFIGENKDLVDPYVQVFFAGQKGKTSVQKSSYEPLWNEQVVFTDLFPPLCKRMKVQIRDSDKVNDVAIGTHFIDLRKISNDGDKGFLPTLGPAWVNMYGSTRNYTLLDEHQDLNEGLGEGVSFRARLMLGLAVEILDTSNPELTSSTEVQVEQATPVSESCTGRMEEFFLFGAFLEASMIDRKNGDKPITFEVTIGNYGNEVDGMSRPLRPRPRKEPGDEEEVDLIQNSSDDEGDEAGDLASVSSTPPMRPQITDRNYFHLPYLERKPCIYIKSWWPDQRRRLYNANIMDHIADKLEEGLNDVQEMIKTEKSYPERRLRGVLEELSCGCHRFLSLSDKDQGRSSRTRLDRERLKSCMRELESMGQQAKSLRAQVKRHTVRDKLRSCQNFLQKLRFLADEPQHSIPDVFIWMMSNNKRIAYARVPSKDLLFSIVEEELGKDCAKVKTLFLKLPGKRGFGSAGWTVQAKLELYLWLGLSKQRKDFLCGLPCGFEEVKAAQGLGLHSFPPISLVYTKKQAFQLRAHMYQARSLFAADSSGLSDPFARVFFINQSQCTEVLNETLCPTWDQMLVFDNLELYGEAHELRDDPPIIVIEIYDQDSMGKADFMGRTFAKPLVKMADEAYCPPRFPPQLEYYQIYRGSATAGDLLAAFELLQIGPSGKADLPPINGPVDMDRGPIMPVPVGIRPVLSKYRVEVLFWGLRDLKRVNLAQVDRPRVDIECAGKGVQSSLIHNYKKNPNFNTLVKWFEVDLPENELLHPPLNIRVVDCRAFGRYTLVGSHAVSSLRRFIYRPPDRSAPNWNTTGEVVVSMEPEEPVKKLETMVKLDATSDAVVKVDVAEDEKERKKKKKKGPSEEPEEEEPDESMLDWWSKYFASIDTMKEQLRQHETSGTDLEEKEEMESAEGLKGPMKSKEKSRAAKEEKKKKNQSPGPGQGSEAPEKKKAKIDELKVYPKELESEFDSFEDWLHTFNLLRGKTGDDEDGSTEEERIVGRFKGSLCVYKVPLPEDVSREAGYDPTYGMFQGIPSNDPINVLVRIYVVRATDLHPADINGKADPYIAIKLGKTDIRDKENYISKQLNPVFGKSFDIEASFPMESMLTVAVYDWDLVGTDDLIGETKIDLENRFYSKHRATCGIAQTYSIHGYNIWRDPMKPSQILTRLCKEGKVDGPHFGPHGRVRVANRVFTGPSEIEDENGQRKPTDEHVALSALRHWEDIPRVGCRLVPEHVETRPLLNPDKPGIEQGRLELWVDMFPMDMPAPGTPLDISPRKPKKYELRVIVWNTDEVVLEDDDFFTGEKSSDIFVRGWLKGQQEDKQDTDVHYHSLTGEGNFNWRYLFPFDYLAAEEKIVMSKKESMFSWDETEYKIPARLTLQIWDADHFSADDFLGAIELDLNRFPRGAKTAKQCTMEMATGEVDVPLVSIFKQKRVKGWWPLLARNENDEFELTGKVEAELHLLTAEEAEKNPVGLARNEPDPLEKPNRPDTAFVWFLNPLKSIKYLICTRYKWLIIKIVLALLGLLMLALFLYSLPGYMVKKLLGA

SEQ ID NO: 8 - DNA, 650 bp, artificial
  Promoter CMV-beta actin = SmCBA
ggtaccctagttattaatagtaatcaattacggggtcattagttcatagcccatatatggagttccgcgttacataacttacggtaaatggcccgcctggctgaccgcccaacgacccccgcccattgacgtcaataatgacgtatgttcccatagtaacgccaatagggactttccattgacgtcaatgggtggactatttacggtaaactgcccacttggcagtacatcaagtgtatcatatgccaagtacgccccctattgacgtcaatgacggtaaatggcccgcctggcattatgcccagtacatgaccttatgggactttcctacttggcagtacatctacgtattagtcatcgctattaccatggtcgaggtgagccccacgttctgcttcactctccccatctcccccccctccccacccccaattttgtatttatttattttttaattattttgtgcagcgatgggggcggggggggggggggggcgcgcgccaggcggggcggggcggggcgaggggcggggcggggcgaggcggagaggtgcggcggcagccaatcagagcggcgcgctccgaaagtttccttttatggcgaggcggcggcggcggcggccctataaaaagcgaagcgcgcggcgggcg

SEQ ID NO: 9 - DNA, 287 bp, artificial
  recombinogenic bridging sequence
ccccgggtgcgcggcgtcggtggtgccggcggggggcgccaggtcgcaggcggtgtagggctccaggcaggcggcgaaggccatgacgtgcgctatgaaggtctgctcctgcacgccgtgaaccaggtgcgcctgcgggccgcgcgcgaacaccgccacgtcctcgcctgcgtgggtctcttcgtccaggggcactgctgactgctgccgatactcggggctcccgctctcgctctcggtaacatccggccgggcgccgtccttgagcacatagcctggaccgtttc

SEQ ID NO: 10 - DNA, 143 bp, artificial
  ITR from AAV2, 5' end
ttggccactccctctctgcgcgctcgctcgctcactgaggccgggcgaccaaaggtcgcccgacgcccgggctttgcccgggcggcctcagtgagcgagcgagcgcgcagagagggagtggccaactccatcactaggggttc

SEQ ID NO: 11 - DNA, 143 bp, artificial
  ITR from AAV2, 3'end
acccctagtgatggagttggccactccctctctgcgcgctcgctcgctcactgaggccgcccgggcaaagcccgggcgtcgggcgacctttggtcgcccggcctcagtgagcgagcgagcgcgcagagagggagtggccaacc

SEQ ID NO: 12 - DNA, 84 bp, artificial
  Splice donor site of the Alkaline Phosphatase
gtaagtatcaaggttacaagacaggtttaaggagaccaatagaaactgggcttgtcgagacagagaagactcttgcgtttctga

SEQ ID NO: 13 - DNA, 49 bp, artificial
  Splice acceptor site of the alkaline phosphatase
taggcacctattggtcttactgacatccactttgcctttctctccacag

SEQ ID NO: 14 - DNA, 20 bp, artificial
  forward primer to amplify a 2676 bp intermediate fragment (nucleotides 27 to 2702) of the otoferlin cDNA
tgtctcagagctccgaggca

SEQ ID NO: 15 - DNA, 22 bp, artificial
  reverse primer to amplify a 2676 bp intermediate fragment (nucleotides 27 to 2702) of the otoferlin cDNA
atcgtggaggaggaactgggca

SEQ ID NO: 16 - DNA, 6907 bp, musc musculus
ttggttgccttggtctctgtgggcagcagcaggaggaggcggcagcagccagagaagagggaggcgtgtgagccacactccaccagcgagcttcttcccgctgctctggaactgcccaggctctccccaccagcatggccctgattgttcacctcaagactgtctcagagctccgaggcaaaggtgaccggattgccaaagtcactttccgagggcagtctttctactcccgggtcctggagaactgcgagggtgtggctgactttgatgagacgttccggtggccagtggccagcagcatcgaccggaatgaagtgttggagattcagattttcaactacagcaaagtcttcagcaacaagctgatagggaccttctgcatggtgctgcagaaagtggtggaggagaatcgggtagaggtgaccgacacgctgatggatgacagcaatgctatcatcaagaccagcctgagcatggaggtccggtatcaggccacagatggcactgtgggcccctgggatgatggagacttcctgggagatgaatccctccaggaggagaaggacagccaggagacagatgggctgctacctggttcccgacccagcacccggatatctggcgagaagagctttcgcagcaaaggcagagagaagaccaagggaggcagagatggcgagcacaaagcgggaaggagtgtgttctcggccatgaaactcggcaaaactcggtcccacaaagaggagccccaaagacaagatgagccagcagtgctggagatggaggacctggaccacctagccattcagctgggggatgggctggatcctgactccgtgtctctagcctcggtcaccgctctcaccagcaatgtctccaacaaacggtctaagccagatattaagatggagcccagtgctggaaggcccatggattaccaggtcagcatcacagtgattgaggctcggcagctggtgggcttgaacatggaccctgtggtgtgtgtggaggtgggtgatgacaagaaatacacgtcaatgaaggagtccacaaactgcccttactacaacgagtactttgtcttcgacttccatgtctctcctgatgtcatgtttgacaagatcatcaagatctcggttatccattctaagaacctgcttcggagcggcaccctggtgggttccttcaaaatggatgtggggactgtgtattcccagcctgaacaccagttccatcacaaatgggccatcctgtcagaccccgatgacatctctgctgggttgaagggttatgtaaagtgtgatgtcgctgtggtgggcaagggagacaacatcaagacaccccacaaggccaacgagacggatgaggacgacattgaagggaacttgctgctccccgagggcgtgccccccgaacggcagtgggcacggttctatgtgaaaatttaccgagcagagggactgccccggatgaacacaagcctcatggccaacgtgaagaaggcgttcatcggtgagaacaaggacctcgtcgacccctatgtgcaagtcttctttgctggacaaaagggcaaaacatcagtgcagaagagcagctatgagccgctatggaatgagcaggtcgtcttcacagacttgttccccccactctgcaaacgcatgaaggtgcagatccgggactctgacaaggtcaatgatgtggccatcggcacccacttcatcgacctgcgcaagatttccaacgatggagacaaaggcttcctgcctaccctcggtccagcctgggtgaacatgtacggctccacgcgcaactacacactgctggacgagcaccaggacttgaatgaaggcctgggggagggtgtgtccttccgggcccgcctcatgttgggactagctgtggagatcctggacacctccaacccagagctcaccagctccacggaggtgcaggtggagcaggccacgcctgtctcggagagctgcacagggagaatggaagaattttttctatttggagccttcttggaagcctcaatgattgaccggaaaaatggggacaagccaattacctttgaggtgaccataggaaactacggcaatgaagtcgatggtatgtcccggcccctgaggcctcggccccggaaagagcctggggatgaagaagaggtagacctgattcagaactccagtgacgatgaaggtgacgaagccggggacctggcctcggtgtcctccaccccacctatgcggccccagatcacggacaggaactatttccacctgccctacctggagcgcaagccctgcatctatatcaagagctggtggcctgaccagaggcggcgcctctacaatgccaacatcatggatcacattgctgacaagctggaagaaggcctgaatgatgtacaggagatgatcaaaacggagaagtcctacccggagcgccgcctgcggggtgtgctagaggaactcagctgtggctgccaccgcttcctctccctctcggacaaggaccagggccgctcgtcccgcaccaggctggatcgagagcgtcttaagtcctgtatgagggagttggagagcatgggacagcaggccaagagcctgagggctcaggtgaagcggcacactgttcgggacaagctgaggtcatgccagaactttctgcagaagctacgcttcctggcggatgagccccagcacagcattcctgatgtgttcatttggatgatgagcaacaacaaacgtatcgcctatgcccgcgtgccttccaaagacctgctcttctccatcgtggaggaggaactgggcaaggactgcgccaaagtcaagaccctcttcctgaagctgccagggaagaggggcttcggctcggcaggctggacagtacaggccaagctggagctctacctgtggctgggcctcagcaagcagcgaaaggacttcctgtgtggtctgccctgtggcttcgaggaggtcaaggcagcccaaggcctgggcctgcattcctttccgcccatcagcctagtctacaccaagaagcaagccttccagctccgagcacacatgtatcaggcccgaagcctctttgctgctgacagcagtgggctctctgatccctttgcccgtgtcttcttcatcaaccagagccaatgcactgaggttctaaacgagacactgtgtcccacctgggaccagatgctggtatttgacaacctggagctgtacggtgaagctcacgagttacgagatgatccccccatcattgtcattgaaatctacgaccaggacagcatgggcaaagccgacttcatgggccggaccttcgccaagcccctggtgaagatggcagatgaagcatactgcccacctcgcttcccgccgcagcttgagtactaccagatctaccgaggcagtgccactgccggagacctactggctgccttcgagctgctgcagattgggccatcagggaaggctgacctgccacccatcaatggcccagtggacatggacagagggcccatcatgcctgtgcccgtgggaatccggccagtgctcagcaagtaccgagtggaggtgctgttctggggcctgagggacctaaagagggtgaacctggcccaggtggaccgaccacgggtggacatcgagtgtgcaggaaagggggtacaatcctccctgattcacaattataagaagaaccccaacttcaacacgctggtcaagtggtttgaagtggacctcccggagaatgagctcctgcacccacccttgaacatccgagtggtagattgccgggcctttggacgatacaccctggtgggttcccacgcagtcagctcactgaggcgcttcatctaccgacctccagaccgctcagcccccaactggaacaccacaggggaggttgtagtaagcatggagcctgaggagccagttaagaagctggagaccatggtgaaactggatgcgacttctgatgctgtggtcaaggtggatgtggctgaagatgagaaggaaaggaagaagaagaaaaagaaaggcccgtcagaggagccagaggaggaagagcccgatgagagcatgctggattggtggtccaagtacttcgcctccatcgacacaatgaaggagcaacttcgacaacatgagacctctggaactgacttggaagagaaggaagagatggaaagcgctgagggcctgaagggaccaatgaagagcaaggagaagtccagagctgcaaaggaggagaaaaagaagaaaaaccagagccctggccctggccagggatcggaggctcctgagaagaagaaagccaagatcgatgagcttaaggtgtaccccaaggagctggaatcggagtttgacagctttgaggactggctgcacaccttcaacctgttgaggggcaagacgggagatgatgaggatggctccacagaggaggagcgcatagtaggccgattcaagggctccctctgtgtgtacaaagtgccactcccagaagatgtatctcgagaagctggctatgatcccacctatggaatgttccagggcatcccaagcaatgaccccatcaatgtgctggtccgaatctatgtggtccgggccacagacctgcacccggccgacatcaatggcaaagctgacccctatattgccatcaagttaggcaagaccgacatccgagacaaggagaactacatctccaagcagctcaaccctgtgtttgggaagtcctttgacattgaggcctccttccccatggagtccatgttgacagtggccgtgtacgactgggatctggtgggcactgatgacctcatcggagaaaccaagattgacctggaaaaccgcttctacagcaagcatcgcgccacctgcggcatcgcacagacctattccatacatggctacaatatctggagggaccccatgaagcccagccagatcctgacacgcctctgtaaagagggcaaagtggacggcccccactttggtccccatgggagagtgagggttgccaaccgtgtcttcacggggccttcagaaatagaggatgagaatggtcagaggaagcccacagatgagcacgtggcactgtctgctctgagacactgggaggacatcccccgggtgggctgccgccttgtgccggaacacgtggagaccaggccgctgctcaaccctgacaagccaggcattgagcagggccgcctggagctgtgggtggacatgttccccatggacatgccagcccctgggacacctctggatatatcccccaggaaacccaagaagtacgagctgcgggtcatcgtgtggaacacagacgaggtggtcctggaagacgatgatttcttcacgggagagaagtccagtgacatttttgtgagggggtggctgaagggccagcaggaggacaaacaggacacagatgtccactatcactccctcacgggggagggcaacttcaactggagatacctcttccccttcgactacctagcggccgaagagaagatcgttatgtccaaaaaggagtctatgttctcctgggatgagacggagtacaagatccctgcgcggctcaccctgcagatctgggacgctgaccacttctcggctgacgacttcctgggggctatcgagctggacctgaaccggttcccgaggggcgctaagacagccaagcagtgcaccatggagatggccaccggggaggtggacgtacccctggtttccatctttaaacagaaacgtgtcaaaggctggtggcccctcctggcccgcaatgagaatgatgagtttgagctcacaggcaaagtggaggcggagctacacctactcacggcagaggaggcagagaagaaccctgtgggcctggctcgcaatgaacctgatcccctagaaaaacccaaccggcctgacacggcattcgtctggttcctgaacccactcaaatctatcaagtacctcatctgcacccggtacaagtggctgatcatcaagatcgtgctggcgctgctggggctgctcatgctggccctcttcctttacagcctcccaggctacatggtcaagaagctcctaggggcctgaagtgtgccccaccccagcccgctccagcatccctccaggggctgctgcgtattttgccttccctcacctggactctctcccaactccctgaggagccctcccacgcctgccagccttgagcaagacacctgcttgctggacttcatccccaccccacacccaaactgttgcttgcctgatcttgtcccaggcctgcctggggtttggggcacagttggcctccaaaaccagataccctcttgtctaaagtaccaggttcctctgcccaaccccaagagtggtagtggcccaaccctccctgtgctttccaaatcttgtcttaaggcaccagtgaaattaaccaagaaacgcggagcaatgcccaaggctctgatgagtaggaacacgtggaaagcaccaggaatgccagcagaggcgaggcggcacacctctctgcagagcatccaggccgagcggcgggcagcggccagctgcttctgcgcatgctctcctcttggctctgcttctttctcacagtcacagtcacttcacagcttagccttgggcttcccatcacttccaggggtgcctctgccttggccagtgtgtgtcagctagtacacaagctccaagtgtgaatcaggtgtactggccgtcctgaagactgactgccctgtccttcctgccgacagccacacccgagtgtacacttaaagcggtgcccttctgcctctgtgggcctgctggctgctgttcctttcttgagtgtgattttttttttctctccctcaataaaataaatcaaactctgagac

SEQ ID NO: 17 - DNA, 7009 bp, artificial
  pTR22-ITR-SmCBA-5'cDNA-otof-SD-RH-ITR
aggggggggggggggggggttggccactccctctctgcgcgctcgctcgctcactgaggccgggcgaccaaaggtcgcccgacgcccgggctttgcccgggcggcctcagtgagcgagcgagcgcgcagagagggagtggccaactccatcactaggggttcctcagatctggcgcgcccaattcggtaccctagttattaatagtaatcaattacggggtcattagttcatagcccatatatggagttccgcgttacataacttacggtaaatggcccgcctggctgaccgcccaacgacccccgcccattgacgtcaataatgacgtatgttcccatagtaacgccaatagggactttccattgacgtcaatgggtggactatttacggtaaactgcccacttggcagtacatcaagtgtatcatatgccaagtacgccccctattgacgtcaatgacggtaaatggcccgcctggcattatgcccagtacatgaccttatgggactttcctacttggcagtacatctacgtattagtcatcgctattaccatggtcgaggtgagccccacgttctgcttcactctccccatctcccccccctccccacccccaattttgtatttatttattttttaattattttgtgcagcgatgggggcggggggggggggggggcgcgcgccaggcggggcggggcggggcgaggggcggggcggggcgaggcggagaggtgcggcggcagccaatcagagcggcgcgctccgaaagtttccttttatggcgaggcggcggcggcggcggccctataaaaagcgaagcgcgcggcgggcgggagtcgctgcgacgctgccttcgccccgtgccccgctccgccgccgcctcgcgccgcccgccccggctctgactgaccgcgttactcccacaggtgagcgggcgggacggcccttctcctccgggctgtaattagcgcttggtttaatgacggcttgtttcttttctgtggctgcgtgaaagccttgaggggctccgggagctagagcctctgctaaccatgttcatgccttcttctttttcctacagctcctgggcaacgtgctggttattgtgctgtctcatcattttggcaaagaattctagcggccgccaccatggccctgattgttcacctcaagactgtctcagagctccgaggcaaaggtgaccggattgccaaagtcactttccgagggcagtctttctactcccgggtcctggagaactgcgagggtgtggctgactttgatgagacgttccggtggccagtggccagcagcatcgaccggaatgaagtgttggagattcagattttcaactacagcaaagtcttcagcaacaagctgatagggaccttctgcatggtgctgcagaaagtggtggaggagaatcgggtagaggtgaccgacacgctgatggatgacagcaatgctatcatcaagaccagcctgagcatggaggtccggtatcaggccacagatggcactgtgggcccctgggatgatggagacttcctgggagatgaatccctccaggaggagaaggacagccaggagacagatgggctgctacctggttcccgacccagcacccggatatctggcgagaagagctttcgcagcaaaggcagagagaagaccaagggaggcagagatggcgagcacaaagcgggaaggagtgtgttctcggccatgaaactcggcaaaactcggtcccacaaagaggagccccaaagacaagatgagccagcagtgctggagatggaggacctggaccacctagccattcagctgggggatgggctggatcctgactccgtgtctctagcctcggtcaccgctctcaccagcaatgtctccaacaaacggtctaagccagatattaagatggagcccagtgctggaaggcccatggattaccaggtcagcatcacagtgattgaggctcggcagctggtgggcttgaacatggaccctgtggtgtgtgtggaggtgggtgatgacaagaaatacacgtcaatgaaggagtccacaaactgcccttactacaacgagtactttgtcttcgacttccatgtctctcctgatgtcatgtttgacaagatcatcaagatctcggttatccattctaagaacctgcttcggagcggcaccctggtgggttccttcaaaatggatgtggggactgtgtattcccagcctgaacaccagttccatcacaaatgggccatcctgtcagaccccgatgacatctctgctgggttgaagggttatgtaaagtgtgatgtcgctgtggtgggcaagggagacaacatcaagacaccccacaaggccaacgagacggatgaggacgacattgaagggaacttgctgctccccgagggcgtgccccccgaacggcagtgggcacggttctatgtgaaaatttaccgagcagagggactgccccggatgaacacaagcctcatggccaacgtgaagaaggcgttcatcggtgagaacaaggacctcgtcgacccctatgtgcaagtcttctttgctggacaaaagggcaaaacatcagtgcagaagagcagctatgagccgctatggaatgagcaggtcgtcttcacagacttgttccccccactctgcaaacgcatgaaggtgcagatccgggactctgacaaggtcaatgatgtggccatcggcacccacttcatcgacctgcgcaagatttccaacgatggagacaaaggcttcctgcctaccctcggtccagcctgggtgaacatgtacggctccacgcgcaactacacactgctggacgagcaccaggacttgaatgaaggcctgggggagggtgtgtccttccgggcccgcctcatgttgggactagctgtggagatcctggacacctccaacccagagctcaccagctccacggaggtgcaggtggagcaggccacgcctgtctcggagagctgcacagggagaatggaagaattttttctatttggagccttcttggaagcctcaatgattgaccggaaaaatggggacaagccaattacctttgaggtgaccataggaaactacggcaatgaagtcgatggtatgtcccggcccctgaggcctcggccccggaaagagcctggggatgaagaagaggtagacctgattcagaactccagtgacgatgaaggtgacgaagccggggacctggcctcggtgtcctccaccccacctatgcggccccagatcacggacaggaactatttccacctgccctacctggagcgcaagccctgcatctatatcaagagctggtggcctgaccagaggcggcgcctctacaatgccaacatcatggatcacattgctgacaagctggaagaaggcctgaatgatgtacaggagatgatcaaaacggagaagtcctacccggagcgccgcctgcggggtgtgctagaggaactcagctgtggctgccaccgcttcctctccctctcggacaaggaccagggccgctcgtcccgcaccaggctggatcgagagcgtcttaagtcctgtatgagggagttggtaagtatcaaggttacaagacaggtttaaggagaccaatagaaactgggcttgtcgagacagagaagactcttgcgtttctgagctagcccccgggtgcgcggcgtcggtggtgccggcggggggcgccaggtcgcaggcggtgtagggctccaggcaggcggcgaaggccatgacgtgcgctatgaaggtctgctcctgcacgccgtgaaccaggtgcgcctgcgggccgcgcgcgaacaccgccacgtcctcgcctgcgtgggtctcttcgtccaggggcactgctgactgctgccgatactcggggctcccgctctcgctctcggtaacatccggccgggcgccgtccttgagcacatagcctggaccgtttcgtcgactgttaattaagcatgctggggagagatctaggaacccctagtgatggagttggccactccctctctgcgcgctcgctcgctcactgaggccgcccgggcaaagcccgggcgtcgggcgacctttggtcgcccggcctcagtgagcgagcgagcgcgcagagagggagtggccaacccccccccccccccccctgcagccctgcattaatgaatcggccaacgcgcggggagaggcggtttgcgtattgggcgctcttccgcttcctcgctcactgactcgctgcgctcggtcgttcggctgcggcgagcggtatcagctcactcaaaggcggtaatacggttatccacagaatcaggggataacgcaggaaagaacatgtgagcaaaaggccagcaaaaggccaggaaccgtaaaaaggccgcgttgctggcgtttttccataggctccgcccccctgacgagcatcacaaaaatcgacgctcaagtcagaggtggcgaaacccgacaggactataaagataccaggcgtttccccctggaagctccctcgtgcgctctcctgttccgaccctgccgcttaccggatacctgtccgcctttctcccttcgggaagcgtggcgctttctcaatgctcacgctgtaggtatctcagttcggtgtaggtcgttcgctccaagctgggctgtgtgcacgaaccccccgttcagcccgaccgctgcgccttatccggtaactatcgtcttgagtccaacccggtaagacacgacttatcgccactggcagcagccactggtaacaggattagcagagcgaggtatgtaggcggtgctacagagttcttgaagtggtggcctaactacggctacactagaaggacagtatttggtatctgcgctctgctgaagccagttaccttcggaaaaagagttggtagctcttgatccggcaaacaaaccaccgctggtagcggtggtttttttgtttgcaagcagcagattacgcgcagaaaaaaaggatctcaagaagatcctttgatcttttctacggggtctgacgctcagtggaacgaaaactcacgttaagggattttggtcatgagattatcaaaaaggatcttcacctagatccttttaaattaaaaatgaagttttaaatcaatctaaagtatatatgagtaaacttggtctgacagttaccaatgcttaatcagtgaggcacctatctcagcgatctgtctatttcgttcatccatagttgcctgactccccgtcgtgtagataactacgatacgggagggcttaccatctggccccagtgctgcaatgataccgcgagacccacgctcaccggctccagatttatcagcaataaaccagccagccggaagggccgagcgcagaagtggtcctgcaactttatccgcctccatccagtctattaattgttgccgggaagctagagtaagtagttcgccagttaatagtttgcgcaacgttgttgccattgctacaggcatcgtggtgtcacgctcgtcgtttggtatggcttcattcagctccggttcccaacgatcaaggcgagttacatgatcccccatgttgtgcaaaaaagcggttagctccttcggtcctccgatcgttgtcagaagtaagttggccgcagtgttatcactcatggttatggcagcactgcataattctcttactgtcatgccatccgtaagatgcttttctgtgactggtgagtactcaaccaagtcattctgagaatagtgtatgcggcgaccgagttgctcttgcccggcgtcaatacgggataataccgcgccacatagcagaactttaaaagtgctcatcattggaaaacgttcttcggggcgaaaactctcaaggatcttaccgctgttgagatccagttcgatgtaacccactcgtgcacccaactgatcttcagcatcttttactttcaccagcgtttctgggtgagcaaaaacaggaaggcaaaatgccgcaaaaaagggaataagggcgacacggaaatgttgaatactcatactcttcctttttcaatattattgaagcatttatcagggttattgtctcatgagcggatacatatttgaatgtatttagaaaaataaacaaataggggttccgcgcacatttccccgaaaagtgccacctgacgtctaagaaaccattattatcatgacattaacctataaaaataggcgtatcacgaggccctttcgtctcgcgcgtttcggtgatgacggtgaaaacctctgacacatgcagctcccggagacggtcacagcttgtctgtaagcggatgccgggagcagacaagcccgtcagggcgcgtcagcgggtgttggcgggtgtcggggctggcttaactatgcggcatcagagcagattgtactgagagtgcaccatatgcggtgtgaaataccgcacagatgcgtaaggagaaaataccgcatcaggaaattgtaaacgttaatattttgttaaaattcgcgttaaatttttgttaaatcagctcattttttaaccaataggccgaaatcggcaaaatcccttataaatcaaaagaatagaccgagatagggttgagtgttgttccagtttggaacaagagtccactattaaagaacgtggactccaacgtcaaagggcgaaaaaccgtctatcagggcgatggcccactacgtgaaccatcaccctaatcaagttttttggggtcgaggtgccgtaaagcactaaatcggaaccctaaagggagcccccgatttagagcttgacggggaaagccggcgaacgtggcgagaaaggaagggaagaaagcgaaaggagcgggcgctagggcgctggcaagtgtagcggtcacgctgcgcgtaaccaccacacccgccgcgcttaatgcgccgctacagggcgcgtcgcgccattcgccattcaggctacgcaactgttgggaagggcgatcggtgcgggcctcttcgctattacgccaggctgc

SEQ ID NO: 18 - DNA, 7413 bp, artificial
  pTR22-ITR-RH-SA- 3'cDNAerlin-polyA-ITR
aggggggggggggggggggttggccactccctctctgcgcgctcgctcgctcactgaggccgggcgaccaaaggtcgcccgacgcccgggctttgcccgggcggcctcagtgagcgagcgagcgcgcagagagggagtggccaactccatcactaggggttcctcagatctggcgcgcccaattggcttcgaattctagcggccgcccccgggtgcgcggcgtcggtggtgccggcggggggcgccaggtcgcaggcggtgtagggctccaggcaggcggcgaaggccatgacgtgcgctatgaaggtctgctcctgcacgccgtgaaccaggtgcgcctgcgggccgcgcgcgaacaccgccacgtcctcgcctgcgtgggtctcttcgtccaggggcactgctgactgctgccgatactcggggctcccgctctcgctctcggtaacatccggccgggcgccgtccttgagcacatagcctggaccgtttccttaagcgacgcatgctcgcgataggcacctattggtcttactgacatccactttgcctttctctccacaggagagcatgggacagcaggccaagagcctgagggctcaggtgaagcggcacactgttcgggacaagctgaggtcatgccagaactttctgcagaagctacgcttcctggcggatgagccccagcacagcattcctgatgtgttcatttggatgatgagcaacaacaaacgtatcgcctatgcccgcgtgccttccaaagacctgctcttctccatcgtggaggaggaactgggcaaggactgcgccaaagtcaagaccctcttcctgaagctgccagggaagaggggcttcggctcggcaggctggacagtacaggccaagctggagctctacctgtggctgggcctcagcaagcagcgaaaggacttcctgtgtggtctgccctgtggcttcgaggaggtcaaggcagcccaaggcctgggcctgcattcctttccgcccatcagcctagtctacaccaagaagcaagccttccagctccgagcacacatgtatcaggcccgaagcctctttgctgctgacagcagtgggctctctgatccctttgcccgtgtcttcttcatcaaccagagccaatgcactgaggttctaaacgagacactgtgtcccacctgggaccagatgctggtatttgacaacctggagctgtacggtgaagctcacgagttacgagatgatccccccatcattgtcattgaaatctacgaccaggacagcatgggcaaagccgacttcatgggccggaccttcgccaagcccctggtgaagatggcagatgaagcatactgcccacctcgcttcccgccgcagcttgagtactaccagatctaccgaggcagtgccactgccggagacctactggctgccttcgagctgctgcagattgggccatcagggaaggctgacctgccacccatcaatggcccagtggacatggacagagggcccatcatgcctgtgcccgtgggaatccggccagtgctcagcaagtaccgagtggaggtgctgttctggggcctgagggacctaaagagggtgaacctggcccaggtggaccgaccacgggtggacatcgagtgtgcaggaaagggggtacaatcctccctgattcacaattataagaagaaccccaacttcaacacgctggtcaagtggtttgaagtggacctcccggagaatgagctcctgcacccacccttgaacatccgagtggtagattgccgggcctttggacgatacaccctggtgggttcccacgcagtcagctcactgaggcgcttcatctaccgacctccagaccgctcagcccccaactggaacaccacaggggaggttgtagtaagcatggagcctgaggagccagttaagaagctggagaccatggtgaaactggatgcgacttctgatgctgtggtcaaggtggatgtggctgaagatgagaaggaaaggaagaagaagaaaaagaaaggcccgtcagaggagccagaggaggaagagcccgatgagagcatgctggattggtggtccaagtacttcgcctccatcgacacaatgaaggagcaacttcgacaacatgagacctctggaactgacttggaagagaaggaagagatggaaagcgctgagggcctgaagggaccaatgaagagcaaggagaagtccagagctgcaaaggaggagaaaaagaagaaaaaccagagccctggccctggccagggatcggaggctcctgagaagaagaaagccaagatcgatgagcttaaggtgtaccccaaggagctggaatcggagtttgacagctttgaggactggctgcacaccttcaacctgttgaggggcaagacgggagatgatgaggatggctccacagaggaggagcgcatagtaggccgattcaagggctccctctgtgtgtacaaagtgccactcccagaagatgtatctcgagaagctggctatgatcccacctatggaatgttccagggcatcccaagcaatgaccccatcaatgtgctggtccgaatctatgtggtccgggccacagacctgcacccggccgacatcaatggcaaagctgacccctatattgccatcaagttaggcaagaccgacatccgagacaaggagaactacatctccaagcagctcaaccctgtgtttgggaagtcctttgacattgaggcctccttccccatggagtccatgttgacagtggccgtgtacgactgggatctggtgggcactgatgacctcatcggagaaaccaagattgacctggaaaaccgcttctacagcaagcatcgcgccacctgcggcatcgcacagacctattccatacatggctacaatatctggagggaccccatgaagcccagccagatcctgacacgcctctgtaaagagggcaaagtggacggcccccactttggtccccatgggagagtgagggttgccaaccgtgtcttcacggggccttcagaaatagaggatgagaatggtcagaggaagcccacagatgagcacgtggcactgtctgctctgagacactgggaggacatcccccgggtgggctgccgccttgtgccggaacacgtggagaccaggccgctgctcaaccctgacaagccaggcattgagcagggccgcctggagctgtgggtggacatgttccccatggacatgccagcccctgggacacctctggatatatcccccaggaaacccaagaagtacgagctgcgggtcatcgtgtggaacacagacgaggtggtcctggaagacgatgatttcttcacgggagagaagtccagtgacatttttgtgagggggtggctgaagggccagcaggaggacaaacaggacacagatgtccactatcactccctcacgggggagggcaacttcaactggagatacctcttccccttcgactacctagcggccgaagagaagatcgttatgtccaaaaaggagtctatgttctcctgggatgagacggagtacaagatccctgcgcggctcaccctgcagatctgggacgctgaccacttctcggctgacgacttcctgggggctatcgagctggacctgaaccggttcccgaggggcgctaagacagccaagcagtgcaccatggagatggccaccggggaggtggacgtacccctggtttccatctttaaacagaaacgtgtcaaaggctggtggcccctcctggcccgcaatgagaatgatgagtttgagctcacaggcaaagtggaggcggagctacacctactcacggcagaggaggcagagaagaaccctgtgggcctggctcgcaatgaacctgatcccctagaaaaacccaaccggcctgacacggcattcgtctggttcctgaacccactcaaatctatcaagtacctcatctgcacccggtacaagtggctgatcatcaagatcgtgctggcgctgctggggctgctcatgctggccctcttcctttacagcctcccaggctacatggtcaagaagctcctaggggcctgagcggccgcggtaccaagggcgaattctgcagtcgactagagctcgctgatcagcctcgactgtgccttctagttgccagccatctgttgtttgcccctcccccgtgccttccttgaccctggaaggtgccactcccactgtcctttcctaataaaatgaggaaattgcatcgcattgtctgagtaggtgtcattctattctggggggtggggtggggcaggacagcaagggggaggattgggaagacaatagcaggcatgctggggagagatctgaggactagtccgtcgactgttaattaagcatgctggggagagatctaggaacccctagtgatggagttggccactccctctctgcgcgctcgctcgctcactgaggccgcccgggcaaagcccgggcgtcgggcgacctttggtcgcccggcctcagtgagcgagcgagcgcgcagagagggagtggccaacccccccccccccccccctgcagccctgcattaatgaatcggccaacgcgcggggagaggcggtttgcgtattgggcgctcttccgcttcctcgctcactgactcgctgcgctcggtcgttcggctgcggcgagcggtatcagctcactcaaaggcggtaatacggttatccacagaatcaggggataacgcaggaaagaacatgtgagcaaaaggccagcaaaaggccaggaaccgtaaaaaggccgcgttgctggcgtttttccataggctccgcccccctgacgagcatcacaaaaatcgacgctcaagtcagaggtggcgaaacccgacaggactataaagataccaggcgtttccccctggaagctccctcgtgcgctctcctgttccgaccctgccgcttaccggatacctgtccgcctttctcccttcgggaagcgtggcgctttctcaatgctcacgctgtaggtatctcagttcggtgtaggtcgttcgctccaagctgggctgtgtgcacgaaccccccgttcagcccgaccgctgcgccttatccggtaactatcgtcttgagtccaacccggtaagacacgacttatcgccactggcagcagccactggtaacaggattagcagagcgaggtatgtaggcggtgctacagagttcttgaagtggtggcctaactacggctacactagaaggacagtatttggtatctgcgctctgctgaagccagttaccttcggaaaaagagttggtagctcttgatccggcaaacaaaccaccgctggtagcggtggtttttttgtttgcaagcagcagattacgcgcagaaaaaaaggatctcaagaagatcctttgatcttttctacggggtctgacgctcagtggaacgaaaactcacgttaagggattttggtcatgagattatcaaaaaggatcttcacctagatccttttaaattaaaaatgaagttttaaatcaatctaaagtatatatgagtaaacttggtctgacagttaccaatgcttaatcagtgaggcacctatctcagcgatctgtctatttcgttcatccatagttgcctgactccccgtcgtgtagataactacgatacgggagggcttaccatctggccccagtgctgcaatgataccgcgagacccacgctcaccggctccagatttatcagcaataaaccagccagccggaagggccgagcgcagaagtggtcctgcaactttatccgcctccatccagtctattaattgttgccgggaagctagagtaagtagttcgccagttaatagtttgcgcaacgttgttgccattgctacaggcatcgtggtgtcacgctcgtcgtttggtatggcttcattcagctccggttcccaacgatcaaggcgagttacatgatcccccatgttgtgcaaaaaagcggttagctccttcggtcctccgatcgttgtcagaagtaagttggccgcagtgttatcactcatggttatggcagcactgcataattctcttactgtcatgccatccgtaagatgcttttctgtgactggtgagtactcaaccaagtcattctgagaatagtgtatgcggcgaccgagttgctcttgcccggcgtcaatacgggataataccgcgccacatagcagaactttaaaagtgctcatcattggaaaacgttcttcggggcgaaaactctcaaggatcttaccgctgttgagatccagttcgatgtaacccactcgtgcacccaactgatcttcagcatcttttactttcaccagcgtttctgggtgagcaaaaacaggaaggcaaaatgccgcaaaaaagggaataagggcgacacggaaatgttgaatactcatactcttcctttttcaatattattgaagcatttatcagggttattgtctcatgagcggatacatatttgaatgtatttagaaaaataaacaaataggggttccgcgcacatttccccgaaaagtgccacctgacgtctaagaaaccattattatcatgacattaacctataaaaataggcgtatcacgaggccctttcgtctcgcgcgtttcggtgatgacggtgaaaacctctgacacatgcagctcccggagacggtcacagcttgtctgtaagcggatgccgggagcagacaagcccgtcagggcgcgtcagcgggtgttggcgggtgtcggggctggcttaactatgcggcatcagagcagattgtactgagagtgcaccatatgcggtgtgaaataccgcacagatgcgtaaggagaaaataccgcatcaggaaattgtaaacgttaatattttgttaaaattcgcgttaaatttttgttaaatcagctcattttttaaccaataggccgaaatcggcaaaatcccttataaatcaaaagaatagaccgagatagggttgagtgttgttccagtttggaacaagagtccactattaaagaacgtggactccaacgtcaaagggcgaaaaaccgtctatcagggcgatggcccactacgtgaaccatcaccctaatcaagttttttggggtcgaggtgccgtaaagcactaaatcggaaccctaaagggagcccccgatttagagcttgacggggaaagccggcgaacgtggcgagaaaggaagggaagaaagcgaaaggagcgggcgctagggcgctggcaagtgtagcggtcacgctgcgcgtaaccaccacacccgccgcgcttaatgcgccgctacagggcgcgtcgcgccattcgccattcaggctacgcaactgttgggaagggcgatcggtgcgggcctcttcgctattacgccaggctgc

SEQ ID NO: 19 - DNA, 6967 bp, artificial
  pTR22-SmCBA-OtoferlinNT-SD-RH-ITR
aggggggggggggggggggttggccactccctctctgcgcgctcgctcgctcactgaggccgggcgaccaaaggtcgcccgacgcccgggctttgcccgggcggcctcagtgagcgagcgagcgcgcagagagggagtggccaactccatcactaggggttcctcagatctggcgcgcccaattcggtaccctagttattaatagtaatcaattacggggtcattagttcatagcccatatatggagttccgcgttacataacttacggtaaatggcccgcctggctgaccgcccaacgacccccgcccattgacgtcaataatgacgtatgttcccatagtaacgccaatagggactttccattgacgtcaatgggtggactatttacggtaaactgcccacttggcagtacatcaagtgtatcatatgccaagtacgccccctattgacgtcaatgacggtaaatggcccgcctggcattatgcccagtacatgaccttatgggactttcctacttggcagtacatctacgtattagtcatcgctattaccatggtcgaggtgagccccacgttctgcttcactctccccatctcccccccctccccacccccaattttgtatttatttattttttaattattttgtgcagcgatgggggcggggggggggggggggcgcgcgccaggcggggcggggcggggcgaggggcggggcggggcgaggcggagaggtgcggcggcagccaatcagagcggcgcgctccgaaagtttccttttatggcgaggcggcggcggcggcggccctataaaaagcgaagcgcgcggcgggcgggagtcgctgcgacgctgccttcgccccgtgccccgctccgccgccgcctcgcgccgcccgccccggctctgactgaccgcgttactcccacaggtgagcgggcgggacggcccttctcctccgggctgtaattagcgcttggtttaatgacggcttgtttcttttctgtggctgcgtgaaagccttgaggggctccgggagctagagcctctgctaaccatgttcatgccttcttctttttcctacagctcctgggcaacgtgctggttattgtgctgtctcatcattttggcaaagaattctagcggccgccaccatggccttgctcatccacctcaagacagtctcggagctgcggggcaggggcgaccggatcgccaaagtgactttccgagggcaatccttctactctcgggtcctggagaactgtgaggatgtggctgactttgatgagacatttcggtggccggtggccagcagcatcgacagaaatgagatgctggagattcaggttttcaactacagcaaagtcttcagcaacaagctcatcgggaccttccgcatggtgctgcagaaggtggtagaggagagccatgtggaggtgactgacacgctgattgatgacaacaatgctatcatcaagaccagcctgtgcgtggaggtccggtatcaggccactgacggcacagtgggctcctgggacgatggggacttcctgggagatgagtctcttcaagaggaagagaaggacagccaagagacggatggactgctcccaggctcccggcccagctcccggcccccaggagagaagagcttccggagagccgggaggagcgtgttctccgccatgaagctcggcaaaaaccggtctcacaaggaggagccccaaagaccagatgaaccggcggtgctggagatggaagaccttgaccatctggccattcggctaggagatggactggatcccgactcggtgtctctagcctcagtcacagctctcaccactaatgtctccaacaagcgatctaagccagacattaagatggagccaagtgctgggcggcccatggattaccaggtcagcatcacggtgatcgaggcccggcagctggtgggcttgaacatggaccctgtggtgtgcgtggaggtgggtgacgacaagaagtacacatccatgaaggagtccactaactgcccctattacaacgagtacttcgtcttcgacttccatgtctctccggatgtcatgtttgacaagatcatcaagatttcggtgattcactccaagaacctgctgcgcagtggcaccctggtgggctccttcaaaatggacgtgggaaccgtgtactcgcagccagagcaccagttccatcacaagtgggccatcctgtctgaccccgatgacatctcctcggggctgaagggctacgtgaagtgtgacgttgccgtggtgggcaaaggggacaacatcaagacgccccacaaggccaatgagaccgacgaagatgacattgaggggaacttgctgctccccgagggggtgccccccgaacgccagtgggcccggttctatgtgaaaatttaccgagcagaggggctgccccgtatgaacacaagcctcatggccaatgtaaagaaggctttcatcggtgaaaacaaggacctcgtggacccctacgtgcaagtcttctttgctggccagaagggcaagacttcagtgcagaagagcagctatgagcccctgtggaatgagcaggtcgtctttacagacctcttccccccactctgcaaacgcatgaaggtgcagatccgagactcggacaaggtcaacgacgtggccatcggcacccacttcattgacctgcgcaagatttctaatgacggagacaaaggcttcctgcccacactgggcccagcctgggtgaacatgtacggctccacacgtaactacacgctgctggatgagcatcaggacctgaacgagggcctgggggagggtgtgtccttccgggcccggctcctgctgggcctggctgtggagatcgtagacacctccaaccctgagctcaccagctccacagaggtgcaggtggagcaggccacgcccatctcggagagctgtgcaggtaaaatggaagaattctttctctttggagccttcctggaggcctcaatgatcgaccggagaaacggagacaagcccatcacctttgaggtcaccataggcaactatgggaacgaagttgatggcctgtcccggccccagcggcctcggccccggaaggagccgggggatgaggaagaagtagacctgattcagaacgcaagtgatgacgaggccggtgatgccggggacctggcctcagtctcctccactccaccaatgcggccccaggtcaccgacaggaactacttccatctgccctacctggagcgaaagccctgcatctacatcaagagctggtggccggaccagcgccgccgcctctacaatgccaacatcatggaccacattgccgacaagctggaagaaggcctgaacgacatacaggagatgatcaaaacggagaagtcctaccctgagcgtcgcctgcggggcgtcctggaggagctgagctgtggctgctgccgcttcctctccctcgctgacaaggaccagggccactcatcccgcaccaggcttgaccgggagcgcctcaagtcctgcatgagggagctggtaagtatcaaggttacaagacaggtttaaggagaccaatagaaactgggcttgtcgagacagagaagactcttgcgtttctgagctagcccccgggtgcgcggcgtcggtggtgccggcggggggcgccaggtcgcaggcggtgtagggctccaggcaggcggcgaaggccatgacgtgcgctatgaaggtctgctcctgcacgccgtgaaccaggtgcgcctgcgggccgcgcgcgaacaccgccacgtcctcgcctgcgtgggtctcttcgtccaggggcactgctgactgctgccgatactcggggctcccgctctcgctctcggtaacatccggccgggcgccgtccttgagcacatagcctggaccgtttcgtcgactgttaattaagcatgctggggagagatctaggaacccctagtgatggagttggccactccctctctgcgcgctcgctcgctcactgaggccgcccgggcaaagcccgggcgtcgggcgacctttggtcgcccggcctcagtgagcgagcgagcgcgcagagagggagtggccaacccccccccccccccccctgcagccctgcattaatgaatcggccaacgcgcggggagaggcggtttgcgtattgggcgctcttccgcttcctcgctcactgactcgctgcgctcggtcgttcggctgcggcgagcggtatcagctcactcaaaggcggtaatacggttatccacagaatcaggggataacgcaggaaagaacatgtgagcaaaaggccagcaaaaggccaggaaccgtaaaaaggccgcgttgctggcgtttttccataggctccgcccccctgacgagcatcacaaaaatcgacgctcaagtcagaggtggcgaaacccgacaggactataaagataccaggcgtttccccctggaagctccctcgtgcgctctcctgttccgaccctgccgcttaccggatacctgtccgcctttctcccttcgggaagcgtggcgctttctcaatgctcacgctgtaggtatctcagttcggtgtaggtcgttcgctccaagctgggctgtgtgcacgaaccccccgttcagcccgaccgctgcgccttatccggtaactatcgtcttgagtccaacccggtaagacacgacttatcgccactggcagcagccactggtaacaggattagcagagcgaggtatgtaggcggtgctacagagttcttgaagtggtggcctaactacggctacactagaaggacagtatttggtatctgcgctctgctgaagccagttaccttcggaaaaagagttggtagctcttgatccggcaaacaaaccaccgctggtagcggtggtttttttgtttgcaagcagcagattacgcgcagaaaaaaaggatctcaagaagatcctttgatcttttctacggggtctgacgctcagtggaacgaaaactcacgttaagggattttggtcatgagattatcaaaaaggatcttcacctagatccttttaaattaaaaatgaagttttaaatcaatctaaagtatatatgagtaaacttggtctgacagttaccaatgcttaatcagtgaggcacctatctcagcgatctgtctatttcgttcatccatagttgcctgactccccgtcgtgtagataactacgatacgggagggcttaccatctggccccagtgctgcaatgataccgcgagacccacgctcaccggctccagatttatcagcaataaaccagccagccggaagggccgagcgcagaagtggtcctgcaactttatccgcctccatccagtctattaattgttgccgggaagctagagtaagtagttcgccagttaatagtttgcgcaacgttgttgccattgctacaggcatcgtggtgtcacgctcgtcgtttggtatggcttcattcagctccggttcccaacgatcaaggcgagttacatgatcccccatgttgtgcaaaaaagcggttagctccttcggtcctccgatcgttgtcagaagtaagttggccgcagtgttatcactcatggttatggcagcactgcataattctcttactgtcatgccatccgtaagatgcttttctgtgactggtgagtactcaaccaagtcattctgagaatagtgtatgcggcgaccgagttgctcttgcccggcgtcaatacgggataataccgcgccacatagcagaactttaaaagtgctcatcattggaaaacgttcttcggggcgaaaactctcaaggatcttaccgctgttgagatccagttcgatgtaacccactcgtgcacccaactgatcttcagcatcttttactttcaccagcgtttctgggtgagcaaaaacaggaaggcaaaatgccgcaaaaaagggaataagggcgacacggaaatgttgaatactcatactcttcctttttcaatattattgaagcatttatcagggttattgtctcatgagcggatacatatttgaatgtatttagaaaaataaacaaataggggttccgcgcacatttccccgaaaagtgccacctgacgtctaagaaaccattattatcatgacattaacctataaaaataggcgtatcacgaggccctttcgtctcgcgcgtttcggtgatgacggtgaaaacctctgacacatgcagctcccggagacggtcacagcttgtctgtaagcggatgccgggagcagacaagcccgtcagggcgcgtcagcgggtgttggcgggtgtcggggctggcttaactatgcggcatcagagcagattgtactgagagtgcaccatatgcggtgtgaaataccgcacagatgcgtaaggagaaaataccgcatcaggaaattgtaaacgttaatattttgttaaaattcgcgttaaatttttgttaaatcagctcattttttaaccaataggccgaaatcggcaaaatcccttataaatcaaaagaatagaccgagatagggttgagtgttgttccagtttggaacaagagtccactattaaagaacgtggactccaacgtcaaagggcgaaaaaccgtctatcagggcgatggcccactacgtgaaccatcaccctaatcaagttttttggggtcgaggtgccgtaaagcactaaatcggaaccctaaagggagcccccgatttagagcttgacggggaaagccggcgaacgtggcgagaaaggaagggaagaaagcgaaaggagcgggcgctagggcgctggcaagtgtagcggtcacgctgcgcgtaaccaccacacccgccgcgcttaatgcgccgctacagggcgcgtcgcgccattcgccattcaggctacgcaactgttgggaagggcgatcggtgcgggcctcttcgctattacgccaggctgc

SEQ ID NO: 20 - DNA, 7470 bp, artificial
  pTR22-ITR-RH-SA-OtoferlinCT-polyA-ITR
aggggggggggggggggggttggccactccctctctgcgcgctcgctcgctcactgaggccgggcgaccaaaggtcgcccgacgcccgggctttgcccgggcggcctcagtgagcgagcgagcgcgcagagagggagtggccaactccatcactaggggttcctcagatctggcgcgcccaattggcttcgaattctagcggccgcccccgggtgcgcggcgtcggtggtgccggcggggggcgccaggtcgcaggcggtgtagggctccaggcaggcggcgaaggccatgacgtgcgctatgaaggtctgctcctgcacgccgtgaaccaggtgcgcctgcgggccgcgcgcgaacaccgccacgtcctcgcctgcgtgggtctcttcgtccaggggcactgctgactgctgccgatactcggggctcccgctctcgctctcggtaacatccggccgggcgccgtccttgagcacatagcctggaccgtttccttaagcgacgcatgctcgcgataggcacctattggtcttactgacatccactttgcctttctctccacaggaaaacatggggcagcaggccaggatgctgcgggcccaggtgaagcggcacacggtgcgggacaagctgaggctgtgccagaacttcctgcagaagctgcgcttcctggcggacgagccccagcacagcattcccgacatcttcatctggatgatgagcaacaacaagcgtgtcgcctatgcccgtgtgccctccaaggacctgctcttctccatcgtggaggaggagactggcaaggactgcgccaaggtcaagacgctcttccttaagctgccagggaagcggggcttcggctcggcaggctggacagtgcaggccaaggtggagctgtacctgtggctgggcctcagcaaacagcgcaaggagttcctgtgcggcctgccctgtggcttccaggaggtcaaggcagcccagggcctgggcctgcatgccttcccacccgtcagcctggtctacaccaagaagcaggcgttccagctccgagcgcacatgtaccaggcccgcagcctctttgccgccgacagcagcggactctcagacccctttgcccgcgtcttcttcatcaatcagagtcagtgcacagaggtgctgaatgagaccctgtgtcccacctgggaccagatgctggtgttcgacaacctggagctctatggtgaagctcatgagctgagggacgatccgcccatcattgtcattgaaatctatgaccaggattccatgggcaaagctgacttcatgggccggaccttcgccaaacccctggtgaagatggcagacgaggcgtactgcccaccccgcttcccacctcagctcgagtactaccagatctaccgtggcaacgccacagctggagacctgctggcggccttcgagctgctgcagattggaccagcagggaaggctgacctgccccccatcaatggcccggtggacgtggaccgaggtcccatcatgcccgtgcccatgggcatccggcccgtgctcagcaagtaccgagtggaggtgctgttctggggcctacgggacctaaagcgggtgaacctggcccaggtggaccggccacgggtggacatcgagtgtgcagggaagggggtgcagtcgtccctgatccacaattataagaagaaccccaacttcaacaccctcgtcaagtggtttgaagtggacctcccagagaacgagctgctgcacccgcccttgaacatccgtgtggtggactgccgggccttcggtcgctacacactggtgggctcccatgccgtcagctccctgcgacgcttcatctaccggcccccagaccgctcggcccccagctggaacaccacggtcaggcttctccggcgctgccgtgtgctgtgcaatgggggctcctcctctcactccacaggggaggttgtggtgactatggagccagaggtacccatcaagaaactggagaccatggtgaagctggacgcgacttctgaagctgttgtcaaggtggatgtggctgaggaggagaaggagaagaagaagaagaagaagggcactgcggaggagccagaggaggaggagccagacgagagcatgctggactggtggtccaagtactttgcctccattgacaccatgaaggagcaacttcgacaacaagagccctctggaattgacttggaggagaaggaggaagtggacaataccgagggcctgaaggggtcaatgaagggcaaggagaaggcaagggctgccaaagaggagaagaagaagaaaactcagagctctggctctggccaggggtccgaggcccccgagaagaagaaacccaagattgatgagcttaaggtataccccaaagagctggagtccgagtttgataactttgaggactggctgcacactttcaacttgcttcggggcaagaccggggatgatgaggatggctccaccgaggaggagcgcattgtgggacgcttcaagggctccctctgcgtgtacaaagtgccactcccagaggacgtgtcccgggaagccggctacgactccacctacggcatgttccagggcatcccgagcaatgaccccatcaatgtgctggtccgagtctatgtggtccgggccacggacctgcaccctgctgacatcaacggcaaagctgacccctacatcgccatccggctaggcaagactgacatccgcgacaaggagaactacatctccaagcagctcaaccctgtctttgggaagtcctttgacatcgaggcctccttccccatggaatccatgctgacggtggctgtgtatgactgggacctggtgggcactgatgacctcattggggaaaccaagatcgacctggagaaccgcttctacagcaagcaccgcgccacctgcggcatcgcccagacctactccacacatggctacaatatctggcgggaccccatgaagcccagccagatcctgacccgcctctgcaaagacggcaaagtggacggcccccactttgggccccctgggagagtgaaggtggccaaccgcgtcttcactgggccctctgagattgaggacgagaacggtcagaggaagcccacagacgagcatgtggcgctgttggccctgaggcactgggaggacatcccccgcgcaggctgccgcctggtgccagagcatgtggagacgaggccgctgctcaaccccgacaagccgggcatcgagcagggccgcctggagctgtgggtggacatgttccccatggacatgccagcccctgggacgcctctggacatctcacctcggaagcccaagaagtacgagctgcgggtcatcatctggaacacagatgaggtggtcttggaggacgacgacttcttcacaggggagaagtccagtgacatcttcgtgagggggtggctgaagggccagcaggaggacaagcaggacacagacgtccactaccactccctcactggcgagggcaacttcaactggcgctacctgttccccttcgactacctggcggcggaggagaagatcgtcatctccaagaaggagtccatgttctcctgggacgagaccgagtacaagatccccgcgcggctcaccctgcagatctgggatgcggaccacttctccgctgacgacttcctgggggccatcgagctggacctgaaccggttcccgcggggcgcaaagacagccaagcagtgcaccatggagatggccaccggggaggtggacgtgcccctcgtgtccatcttcaagcaaaagcgcgtcaaaggctggtggcccctcctggcccgcaatgagaacgatgagtttgagctcacgggcaaggtggaggctgagctgcatttactgacagcagaggaggcagagaagaacccagtgggcctggcccgcaatgaacctgaccccctagagaaacccaaccggcccgacacgagcttcatctggttcctgaaccctctcaagtcggctcgctacttcttgtggcacacgtatcgctggctgctcctcaaactgttgctgctcctgctgctgctcctcctcctcgccctgttcctctactctgtgcctggctacctggtcaagaaaatcctcggggcctgagcggccgcggtaccaagggcgaattctgcagtcgactagagctcgctgatcagcctcgactgtgccttctagttgccagccatctgttgtttgcccctcccccgtgccttccttgaccctggaaggtgccactcccactgtcctttcctaataaaatgaggaaattgcatcgcattgtctgagtaggtgtcattctattctggggggtggggtggggcaggacagcaagggggaggattgggaagacaatagcaggcatgctggggagagatctgaggactagtccgtcgactgttaattaagcatgctggggagagatctaggaacccctagtgatggagttggccactccctctctgcgcgctcgctcgctcactgaggccgcccgggcaaagcccgggcgtcgggcgacctttggtcgcccggcctcagtgagcgagcgagcgcgcagagagggagtggccaacccccccccccccccccctgcagccctgcattaatgaatcggccaacgcgcggggagaggcggtttgcgtattgggcgctcttccgcttcctcgctcactgactcgctgcgctcggtcgttcggctgcggcgagcggtatcagctcactcaaaggcggtaatacggttatccacagaatcaggggataacgcaggaaagaacatgtgagcaaaaggccagcaaaaggccaggaaccgtaaaaaggccgcgttgctggcgtttttccataggctccgcccccctgacgagcatcacaaaaatcgacgctcaagtcagaggtggcgaaacccgacaggactataaagataccaggcgtttccccctggaagctccctcgtgcgctctcctgttccgaccctgccgcttaccggatacctgtccgcctttctcccttcgggaagcgtggcgctttctcaatgctcacgctgtaggtatctcagttcggtgtaggtcgttcgctccaagctgggctgtgtgcacgaaccccccgttcagcccgaccgctgcgccttatccggtaactatcgtcttgagtccaacccggtaagacacgacttatcgccactggcagcagccactggtaacaggattagcagagcgaggtatgtaggcggtgctacagagttcttgaagtggtggcctaactacggctacactagaaggacagtatttggtatctgcgctctgctgaagccagttaccttcggaaaaagagttggtagctcttgatccggcaaacaaaccaccgctggtagcggtggtttttttgtttgcaagcagcagattacgcgcagaaaaaaaggatctcaagaagatcctttgatcttttctacggggtctgacgctcagtggaacgaaaactcacgttaagggattttggtcatgagattatcaaaaaggatcttcacctagatccttttaaattaaaaatgaagttttaaatcaatctaaagtatatatgagtaaacttggtctgacagttaccaatgcttaatcagtgaggcacctatctcagcgatctgtctatttcgttcatccatagttgcctgactccccgtcgtgtagataactacgatacgggagggcttaccatctggccccagtgctgcaatgataccgcgagacccacgctcaccggctccagatttatcagcaataaaccagccagccggaagggccgagcgcagaagtggtcctgcaactttatccgcctccatccagtctattaattgttgccgggaagctagagtaagtagttcgccagttaatagtttgcgcaacgttgttgccattgctacaggcatcgtggtgtcacgctcgtcgtttggtatggcttcattcagctccggttcccaacgatcaaggcgagttacatgatcccccatgttgtgcaaaaaagcggttagctccttcggtcctccgatcgttgtcagaagtaagttggccgcagtgttatcactcatggttatggcagcactgcataattctcttactgtcatgccatccgtaagatgcttttctgtgactggtgagtactcaaccaagtcattctgagaatagtgtatgcggcgaccgagttgctcttgcccggcgtcaatacgggataataccgcgccacatagcagaactttaaaagtgctcatcattggaaaacgttcttcggggcgaaaactctcaaggatcttaccgctgttgagatccagttcgatgtaacccactcgtgcacccaactgatcttcagcatcttttactttcaccagcgtttctgggtgagcaaaaacaggaaggcaaaatgccgcaaaaaagggaataagggcgacacggaaatgttgaatactcatactcttcctttttcaatattattgaagcatttatcagggttattgtctcatgagcggatacatatttgaatgtatttagaaaaataaacaaataggggttccgcgcacatttccccgaaaagtgccacctgacgtctaagaaaccattattatcatgacattaacctataaaaataggcgtatcacgaggccctttcgtctcgcgcgtttcggtgatgacggtgaaaacctctgacacatgcagctcccggagacggtcacagcttgtctgtaagcggatgccgggagcagacaagcccgtcagggcgcgtcagcgggtgttggcgggtgtcggggctggcttaactatgcggcatcagagcagattgtactgagagtgcaccatatgcggtgtgaaataccgcacagatgcgtaaggagaaaataccgcatcaggaaattgtaaacgttaatattttgttaaaattcgcgttaaatttttgttaaatcagctcattttttaaccaataggccgaaatcggcaaaatcccttataaatcaaaagaatagaccgagatagggttgagtgttgttccagtttggaacaagagtccactattaaagaacgtggactccaacgtcaaagggcgaaaaaccgtctatcagggcgatggcccactacgtgaaccatcaccctaatcaagttttttggggtcgaggtgccgtaaagcactaaatcggaaccctaaagggagcccccgatttagagcttgacggggaaagccggcgaacgtggcgagaaaggaagggaagaaagcgaaaggagcgggcgctagggcgctggcaagtgtagcggtcacgctgcgcgtaaccaccacacccgccgcgcttaatgcgccgctacagggcgcgtcgcgccattcgccattcaggctacgcaactgttgggaagggcgatcggtgcgggcctcttcgctattacgccaggctgc

SEQ ID NO: 21 - DNA, 7470 bp, artificial
  pTR22-ITR-RH-SA-OtoferlinCT-polyA-ITR
aggggggggggggggggggttggccactccctctctgcgcgctcgctcgctcactgaggccgggcgaccaaaggtcgcccgacgcccgggctttgcccgggcggcctcagtgagcgagcgagcgcgcagagagggagtggccaactccatcactaggggttcctcagatctggcgcgcccaattggcttcgaattctagcggccgcccccgggtgcgcggcgtcggtggtgccggcggggggcgccaggtcgcaggcggtgtagggctccaggcaggcggcgaaggccatgacgtgcgctatgaaggtctgctcctgcacgccgtgaaccaggtgcgcctgcgggccgcgcgcgaacaccgccacgtcctcgcctgcgtgggtctcttcgtccaggggcactgctgactgctgccgatactcggggctcccgctctcgctctcggtaacatccggccgggcgccgtccttgagcacatagcctggaccgtttccttaagcgacgcatgctcgcgataggcacctattggtcttactgacatccactttgcctttctctccacaggaaaacatggggcagcaggccaggatgctgcgggcccaggtgaagcggcacacggtgcgggacaagctgaggctgtgccagaacttcctgcagaagctgcgcttcctggcggacgagccccagcacagcattcccgacatcttcatctggatgatgagcaacaacaagcgtgtcgcctatgcccgtgtgccctccaaggacctgctcttctccatcgtggaggaggagactggcaaggactgcgccaaggtcaagacgctcttccttaagctgccagggaagcggggcttcggctcggcaggctggacagtgcaggccaaggtggagctgtacctgtggctgggcctcagcaaacagcgcaaggagttcctgtgcggcctgccctgtggcttccaggaggtcaaggcagcccagggcctgggcctgcatgccttcccacccgtcagcctggtctacaccaagaagcaggcgttccagctccgagcgcacatgtaccaggcccgcagcctctttgccgccgacagcagcggactctcagacccctttgcccgcgtcttcttcatcaatcagagtcagtgcacagaggtgctgaatgagaccctgtgtcccacctgggaccagatgctggtgttcgacaacctggagctctatggtgaagctcatgagctgagggacgatccgcccatcattgtcattgaaatctatgaccaggattccatgggcaaagctgacttcatgggccggaccttcgccaaacccctggtgaagatggcagacgaggcgtactgcccaccccgcttcccacctcagctcgagtactaccagatctaccgtggcaacgccacagctggagacctgctggcggccttcgagctgctgcagattggaccagcagggaaggctgacctgccccccatcaatggcccggtggacgtggaccgaggtcccatcatgcccgtgcccatgggcatccggcccgtgctcagcaagtaccgagtggaggtgctgttctggggcctacgggacctaaagcgggtgaacctggcccaggtggaccggccacgggtggacatcgagtgtgcagggaagggggtgcagtcgtccctgatccacaattataagaagaaccccaacttcaacaccctcgtcaagtggtttgaagtggacctcccagagaacgagctgctgcacccgcccttgaacatccgtgtggtggactgccgggccttcggtcgctacacactggtgggctcccatgccgtcagctccctgcgacgcttcatctaccggcccccagaccgctcggcccccagctggaacaccacggtcaggcttctccggcgctgccgtgtgctgtgcaatgggggctcctcctctcactccacaggggaggttgtggtgactatggagccagaggtacccatcaagaaactggagaccatggtgaagctggacgcgacttctgaagctgttgtcaaggtggatgtggctgaggaggagaaggagaagaagaagaagaagaagggcactgcggaggagccagaggaggaggagccagacgagagcatgctggactggtggtccaagtactttgcctccattgacaccatgaaggagcaacttcgacaacaagagccctctggaattgacttggaggagaaggaggaagtggacaataccgagggcctgaaggggtcaatgaagggcaaggagaaggcaagggctgccaaagaggagaagaagaagaaaactcagagctctggctctggccaggggtccgaggcccccgagaagaagaaacccaagattgatgagcttaaggtataccccaaagagctggagtccgagtttgataactttgaggactggctgcacactttcaacttgcttcggggcaagaccggggatgatgaggatggctccaccgaggaggagcgcattgtgggacgcttcaagggctccctctgcgtgtacaaagtgccactcccagaggacgtgtcccgggaagccggctacgactccacctacggcatgttccagggcatcccgagcaatgaccccatcaatgtgctggtccgagtctatgtggtccgggccacggacctgcaccctgctgacatcaacggcaaagctgacccctacatcgccatccggctaggcaagactgacatccgcgacaaggagaactacatctccaagcagctcaaccctgtctttgggaagtcctttgacatcgaggcctccttccccatggaatccatgctgacggtggctgtgtatgactgggacctggtgggcactgatgacctcattggggaaaccaagatcgacctggagaaccgcttctacagcaagcaccgcgccacctgcggcatcgcccagacctactccacacatggctacaatatctggcgggaccccatgaagcccagccagatcctgacccgcctctgcaaagacggcaaagtggacggcccccactttgggccccctgggagagtgaaggtggccaaccgcgtcttcactgggccctctgagattgaggacgagaacggtcagaggaagcccacagacgagcatgtggcgctgttggccctgaggcactgggaggacatcccccgcgcaggctgccgcctggtgccagagcatgtggagacgaggccgctgctcaaccccgacaagccgggcatcgagcagggccgcctggagctgtgggtggacatgttccccatggacatgccagcccctgggacgcctctggacatctcacctcggaagcccaagaagtacgagctgcgggtcatcatctggaacacagatgaggtggtcttggaggacgacgacttcttcacaggggagaagtccagtgacatcttcgtgagggggtggctgaagggccagcaggaggacaagcaggacacagacgtccactaccactccctcactggcgagggcaacttcaactggcgctacctgttccccttcgactacctggcggcggaggagaagatcgtcatctccaagaaggagtccatgttctcctgggacgagaccgagtacaagatccccgcgcggctcaccctgcagatctgggatgcggaccacttctccgctgacgacttcctgggggccatcgagctggacctgaaccggttcccgcggggcgcaaagacagccaagcagtgcaccatggagatggccaccggggaggtggacgtgcccctcgtgtccatcttcaagcaaaagcgcgtcaaaggctggtggcccctcctggcccgcaatgagaacgatgagtttgagctcacgggcaaggtggaggctgagctgcatttactgacagcagaggaggcagagaagaacccagtgggcctggcccgcaatgaacctgaccccctagagaaacccaaccggcccgacacggccttcgtctggttcctcaaccctctcaagtccatcaagtacctcatctgcacccggtacaagtggctcatcatcaagatcgtgctggcgctgttggggctgctcatgttggggctcttcctctacagcctccctggctacatggtcaaaaagctccttggggcatgagcggccgcggtaccaagggcgaattctgcagtcgactagagctcgctgatcagcctcgactgtgccttctagttgccagccatctgttgtttgcccctcccccgtgccttccttgaccctggaaggtgccactcccactgtcctttcctaataaaatgaggaaattgcatcgcattgtctgagtaggtgtcattctattctggggggtggggtggggcaggacagcaagggggaggattgggaagacaatagcaggcatgctggggagagatctgaggactagtccgtcgactgttaattaagcatgctggggagagatctaggaacccctagtgatggagttggccactccctctctgcgcgctcgctcgctcactgaggccgcccgggcaaagcccgggcgtcgggcgacctttggtcgcccggcctcagtgagcgagcgagcgcgcagagagggagtggccaacccccccccccccccccctgcagccctgcattaatgaatcggccaacgcgcggggagaggcggtttgcgtattgggcgctcttccgcttcctcgctcactgactcgctgcgctcggtcgttcggctgcggcgagcggtatcagctcactcaaaggcggtaatacggttatccacagaatcaggggataacgcaggaaagaacatgtgagcaaaaggccagcaaaaggccaggaaccgtaaaaaggccgcgttgctggcgtttttccataggctccgcccccctgacgagcatcacaaaaatcgacgctcaagtcagaggtggcgaaacccgacaggactataaagataccaggcgtttccccctggaagctccctcgtgcgctctcctgttccgaccctgccgcttaccggatacctgtccgcctttctcccttcgggaagcgtggcgctttctcaatgctcacgctgtaggtatctcagttcggtgtaggtcgttcgctccaagctgggctgtgtgcacgaaccccccgttcagcccgaccgctgcgccttatccggtaactatcgtcttgagtccaacccggtaagacacgacttatcgccactggcagcagccactggtaacaggattagcagagcgaggtatgtaggcggtgctacagagttcttgaagtggtggcctaactacggctacactagaaggacagtatttggtatctgcgctctgctgaagccagttaccttcggaaaaagagttggtagctcttgatccggcaaacaaaccaccgctggtagcggtggtttttttgtttgcaagcagcagattacgcgcagaaaaaaaggatctcaagaagatcctttgatcttttctacggggtctgacgctcagtggaacgaaaactcacgttaagggattttggtcatgagattatcaaaaaggatcttcacctagatccttttaaattaaaaatgaagttttaaatcaatctaaagtatatatgagtaaacttggtctgacagttaccaatgcttaatcagtgaggcacctatctcagcgatctgtctatttcgttcatccatagttgcctgactccccgtcgtgtagataactacgatacgggagggcttaccatctggccccagtgctgcaatgataccgcgagacccacgctcaccggctccagatttatcagcaataaaccagccagccggaagggccgagcgcagaagtggtcctgcaactttatccgcctccatccagtctattaattgttgccgggaagctagagtaagtagttcgccagttaatagtttgcgcaacgttgttgccattgctacaggcatcgtggtgtcacgctcgtcgtttggtatggcttcattcagctccggttcccaacgatcaaggcgagttacatgatcccccatgttgtgcaaaaaagcggttagctccttcggtcctccgatcgttgtcagaagtaagttggccgcagtgttatcactcatggttatggcagcactgcataattctcttactgtcatgccatccgtaagatgcttttctgtgactggtgagtactcaaccaagtcattctgagaatagtgtatgcggcgaccgagttgctcttgcccggcgtcaatacgggataataccgcgccacatagcagaactttaaaagtgctcatcattggaaaacgttcttcggggcgaaaactctcaaggatcttaccgctgttgagatccagttcgatgtaacccactcgtgcacccaactgatcttcagcatcttttactttcaccagcgtttctgggtgagcaaaaacaggaaggcaaaatgccgcaaaaaagggaataagggcgacacggaaatgttgaatactcatactcttcctttttcaatattattgaagcatttatcagggttattgtctcatgagcggatacatatttgaatgtatttagaaaaataaacaaataggggttccgcgcacatttccccgaaaagtgccacctgacgtctaagaaaccattattatcatgacattaacctataaaaataggcgtatcacgaggccctttcgtctcgcgcgtttcggtgatgacggtgaaaacctctgacacatgcagctcccggagacggtcacagcttgtctgtaagcggatgccgggagcagacaagcccgtcagggcgcgtcagcgggtgttggcgggtgtcggggctggcttaactatgcggcatcagagcagattgtactgagagtgcaccatatgcggtgtgaaataccgcacagatgcgtaaggagaaaataccgcatcaggaaattgtaaacgttaatattttgttaaaattcgcgttaaatttttgttaaatcagctcattttttaaccaataggccgaaatcggcaaaatcccttataaatcaaaagaatagaccgagatagggttgagtgttgttccagtttggaacaagagtccactattaaagaacgtggactccaacgtcaaagggcgaaaaaccgtctatcagggcgatggcccactacgtgaaccatcaccctaatcaagttttttggggtcgaggtgccgtaaagcactaaatcggaaccctaaagggagcccccgatttagagcttgacggggaaagccggcgaacgtggcgagaaaggaagggaagaaagcgaaaggagcgggcgctagggcgctggcaagtgtagcggtcacgctgcgcgtaaccaccacacccgccgcgcttaatgcgccgctacagggcgcgtcgcgccattcgccattcaggctacgcaactgttgggaagggcgatcggtgcgggcctcttcgctattacgccaggctgc

SEQ ID NO: 22 - DNA, 6973 bp, homo sapiens
atcggaggggggtcgggaggaggaggaggaggcagcggcagagaagagagaggcgtgtgagccgtgctccaccggctagctccttcccgctgctcctgcctggcagtgccaggcagcccacaccagcatggccttgctcatccacctcaagacagtctcggagctgcggggcaggggcgaccggatcgccaaagtgactttccgagggcaatccttctactctcgggtcctggagaactgtgaggatgtggctgactttgatgagacatttcggtggccggtggccagcagcatcgacagaaatgagatgctggagattcaggttttcaactacagcaaagtcttcagcaacaagctcatcgggaccttccgcatggtgctgcagaaggtggtagaggagagccatgtggaggtgactgacacgctgattgatgacaacaatgctatcatcaagaccagcctgtgcgtggaggtccggtatcaggccactgacggcacagtgggctcctgggacgatggggacttcctgggagatgagtctcttcaagaggaagagaaggacagccaagagacggatggactgctcccaggctcccggcccagctcccggcccccaggagagaagagcttccggagagccgggaggagcgtgttctccgccatgaagctcggcaaaaaccggtctcacaaggaggagccccaaagaccagatgaaccggcggtgctggagatggaagaccttgaccatctggccattcggctaggagatggactggatcccgactcggtgtctctagcctcagtcacagctctcaccactaatgtctccaacaagcgatctaagccagacattaagatggagccaagtgctgggcggcccatggattaccaggtcagcatcacggtgatcgaggcccggcagctggtgggcttgaacatggaccctgtggtgtgcgtggaggtgggtgacgacaagaagtacacatccatgaaggagtccactaactgcccctattacaacgagtacttcgtcttcgacttccatgtctctccggatgtcatgtttgacaagatcatcaagatttcggtgattcactccaagaacctgctgcgcagtggcaccctggtgggctccttcaaaatggacgtgggaaccgtgtactcgcagccagagcaccagttccatcacaagtgggccatcctgtctgaccccgatgacatctcctcggggctgaagggctacgtgaagtgtgacgttgccgtggtgggcaaaggggacaacatcaagacgccccacaaggccaatgagaccgacgaagatgacattgaggggaacttgctgctccccgagggggtgccccccgaacgccagtgggcccggttctatgtgaaaatttaccgagcagaggggctgccccgtatgaacacaagcctcatggccaatgtaaagaaggctttcatcggtgaaaacaaggacctcgtggacccctacgtgcaagtcttctttgctggccagaagggcaagacttcagtgcagaagagcagctatgagcccctgtggaatgagcaggtcgtctttacagacctcttccccccactctgcaaacgcatgaaggtgcagatccgagactcggacaaggtcaacgacgtggccatcggcacccacttcattgacctgcgcaagatttctaatgacggagacaaaggcttcctgcccacactgggcccagcctgggtgaacatgtacggctccacacgtaactacacgctgctggatgagcatcaggacctgaacgagggcctgggggagggtgtgtccttccgggcccggctcctgctgggcctggctgtggagatcgtagacacctccaaccctgagctcaccagctccacagaggtgcaggtggagcaggccacgcccatctcggagagctgtgcaggtaaaatggaagaattctttctctttggagccttcctggaggcctcaatgatcgaccggagaaacggagacaagcccatcacctttgaggtcaccataggcaactatgggaacgaagttgatggcctgtcccggccccagcggcctcggccccggaaggagccgggggatgaggaagaagtagacctgattcagaacgcaagtgatgacgaggccggtgatgccggggacctggcctcagtctcctccactccaccaatgcggccccaggtcaccgacaggaactacttccatctgccctacctggagcgaaagccctgcatctacatcaagagctggtggccggaccagcgccgccgcctctacaatgccaacatcatggaccacattgccgacaagctggaagaaggcctgaacgacatacaggagatgatcaaaacggagaagtcctaccctgagcgtcgcctgcggggcgtcctggaggagctgagctgtggctgctgccgcttcctctccctcgctgacaaggaccagggccactcatcccgcaccaggcttgaccgggagcgcctcaagtcctgcatgagggagctggaaaacatggggcagcaggccaggatgctgcgggcccaggtgaagcggcacacggtgcgggacaagctgaggctgtgccagaacttcctgcagaagctgcgcttcctggcggacgagccccagcacagcattcccgacatcttcatctggatgatgagcaacaacaagcgtgtcgcctatgcccgtgtgccctccaaggacctgctcttctccatcgtggaggaggagactggcaaggactgcgccaaggtcaagacgctcttccttaagctgccagggaagcggggcttcggctcggcaggctggacagtgcaggccaaggtggagctgtacctgtggctgggcctcagcaaacagcgcaaggagttcctgtgcggcctgccctgtggcttccaggaggtcaaggcagcccagggcctgggcctgcatgccttcccacccgtcagcctggtctacaccaagaagcaggcgttccagctccgagcgcacatgtaccaggcccgcagcctctttgccgccgacagcagcggactctcagacccctttgcccgcgtcttcttcatcaatcagagtcagtgcacagaggtgctgaatgagaccctgtgtcccacctgggaccagatgctggtgttcgacaacctggagctctatggtgaagctcatgagctgagggacgatccgcccatcattgtcattgaaatctatgaccaggattccatgggcaaagctgacttcatgggccggaccttcgccaaacccctggtgaagatggcagacgaggcgtactgcccaccccgcttcccacctcagctcgagtactaccagatctaccgtggcaacgccacagctggagacctgctggcggccttcgagctgctgcagattggaccagcagggaaggctgacctgccccccatcaatggcccggtggacgtggaccgaggtcccatcatgcccgtgcccatgggcatccggcccgtgctcagcaagtaccgagtggaggtgctgttctggggcctacgggacctaaagcgggtgaacctggcccaggtggaccggccacgggtggacatcgagtgtgcagggaagggggtgcagtcgtccctgatccacaattataagaagaaccccaacttcaacaccctcgtcaagtggtttgaagtggacctcccagagaacgagctgctgcacccgcccttgaacatccgtgtggtggactgccgggccttcggtcgctacacactggtgggctcccatgccgtcagctccctgcgacgcttcatctaccggcccccagaccgctcggcccccagctggaacaccacggtcaggcttctccggcgctgccgtgtgctgtgcaatgggggctcctcctctcactccacaggggaggttgtggtgactatggagccagaggtacccatcaagaaactggagaccatggtgaagctggacgcgacttctgaagctgttgtcaaggtggatgtggctgaggaggagaaggagaagaagaagaagaagaagggcactgcggaggagccagaggaggaggagccagacgagagcatgctggactggtggtccaagtactttgcctccattgacaccatgaaggagcaacttcgacaacaagagccctctggaattgacttggaggagaaggaggaagtggacaataccgagggcctgaaggggtcaatgaagggcaaggagaaggcaagggctgccaaagaggagaagaagaagaaaactcagagctctggctctggccaggggtccgaggcccccgagaagaagaaacccaagattgatgagcttaaggtataccccaaagagctggagtccgagtttgataactttgaggactggctgcacactttcaacttgcttcggggcaagaccggggatgatgaggatggctccaccgaggaggagcgcattgtgggacgcttcaagggctccctctgcgtgtacaaagtgccactcccagaggacgtgtcccgggaagccggctacgactccacctacggcatgttccagggcatcccgagcaatgaccccatcaatgtgctggtccgagtctatgtggtccgggccacggacctgcaccctgctgacatcaacggcaaagctgacccctacatcgccatccggctaggcaagactgacatccgcgacaaggagaactacatctccaagcagctcaaccctgtctttgggaagtcctttgacatcgaggcctccttccccatggaatccatgctgacggtggctgtgtatgactgggacctggtgggcactgatgacctcattggggaaaccaagatcgacctggagaaccgcttctacagcaagcaccgcgccacctgcggcatcgcccagacctactccacacatggctacaatatctggcgggaccccatgaagcccagccagatcctgacccgcctctgcaaagacggcaaagtggacggcccccactttgggccccctgggagagtgaaggtggccaaccgcgtcttcactgggccctctgagattgaggacgagaacggtcagaggaagcccacagacgagcatgtggcgctgttggccctgaggcactgggaggacatcccccgcgcaggctgccgcctggtgccagagcatgtggagacgaggccgctgctcaaccccgacaagccgggcatcgagcagggccgcctggagctgtgggtggacatgttccccatggacatgccagcccctgggacgcctctggacatctcacctcggaagcccaagaagtacgagctgcgggtcatcatctggaacacagatgaggtggtcttggaggacgacgacttcttcacaggggagaagtccagtgacatcttcgtgagggggtggctgaagggccagcaggaggacaagcaggacacagacgtccactaccactccctcactggcgagggcaacttcaactggcgctacctgttccccttcgactacctggcggcggaggagaagatcgtcatctccaagaaggagtccatgttctcctgggacgagaccgagtacaagatccccgcgcggctcaccctgcagatctgggatgcggaccacttctccgctgacgacttcctgggggccatcgagctggacctgaaccggttcccgcggggcgcaaagacagccaagcagtgcaccatggagatggccaccggggaggtggacgtgcccctcgtgtccatcttcaagcaaaagcgcgtcaaaggctggtggcccctcctggcccgcaatgagaacgatgagtttgagctcacgggcaaggtggaggctgagctgcatttactgacagcagaggaggcagagaagaacccagtgggcctggcccgcaatgaacctgaccccctagagaaacccaaccggcccgacacggccttcgtctggttcctcaaccctctcaagtccatcaagtacctcatctgcacccggtacaagtggctcatcatcaagatcgtgctggcgctgttggggctgctcatgttggggctcttcctctacagcctccctggctacatggtcaaaaagctccttggggcatgaaggccgccagctcccgccagccgctccccagccctgccgcatttcctttcagtggcttggactctttcccatctcccctggggagcctgaggagcccagcgtccactcttcatgccttgggccgagcctgcctcctgcttgcgggggccgcctgtcctcactgccccaggctgcggcttgcccagtcccgcccctctgacccctgcctgtgggctggggagccttggatggggtggggacctggaatgggtctctcttgccccacctggctgaggcgccacccttcttcaggcccaggctccagaggaagactcctgaaaccctccccaggtcttccaagtacaggattgaagctttagtgaaattaaccaaggaccatgggtcagtgcccagggctttaaaaagaatgaacgagcaaaaggtatccccgccgtgacccctgcagatagcaccggtctttgatccgcagcaggggccagaccctgcccacaagtcccagcgcggctgcttctgccactgctgggctccacttggctcctctcacttcccagggggtcgcctgtcctgcctgtgggtttccatggcttcccagagctccctctgccccagccagcgcctccaggcccagctgaggagctgtgagaagcagcagaggggactccccatcccgggcacaccctgtcctcccacccctgcccccttgcccttccagccctttcagctgcagctgggagctggcccgtcaagtgctgcccctgcctgtgtctgggtttctgttggctgtttttcttttcttgagtggtgatttttctctaaataaaagaagtcaagcactgaaaaaaaaaaaaaaaa

SEQ ID NO: 23 - DNA, 3318 bp, homo sapiens
ctgccagggaagcggggcttcggctcggcaggctggacagtgcaggccaaggtggagctgtacctgtggctgggcctcagcaaacagcgcaaggagttcctgtgcggcctgccctgtggcttccaggaggtcaaggcagcccagggcctgggcctgcatgccttcccacccgtcagcctggtctacaccaagaagcaggcgttccagctccgagcgcacatgtaccaggcccgcagcctctttgccgccgacagcagcggactctcagacccctttgcccgcgtcttcttcatcaatcagagtcagtgcacagaggtgctgaatgagaccctgtgtcccacctgggaccagatgctggtgttcgacaacctggagctctatggtgaagctcatgagctgagggacgatccgcccatcattgtcattgaaatctatgaccaggattccatgggcaaagctgacttcatgggccggaccttcgccaaacccctggtgaagatggcagacgaggcgtactgcccaccccgcttcccacctcagctcgagtactaccagatctaccgtggcaacgccacagctggagacctgctggcggccttcgagctgctgcagattggaccagcagggaaggctgacctgccccccatcaatggcccggtggacgtggaccgaggtcccatcatgcccgtgcccatgggcatccggcccgtgctcagcaagtaccgagtggaggtgctgttctggggcctacgggacctaaagcgggtgaacctggcccaggtggaccggccacgggtggacatcgagtgtgcagggaagggggtgcagtcgtccctgatccacaattataagaagaaccccaacttcaacaccctcgtcaagtggtttgaagtggacctcccagagaacgagctgctgcacccgcccttgaacatccgtgtggtggactgccgggccttcggtcgctacacactggtgggctcccatgccgtcagctccctgcgacgcttcatctaccggcccccagaccgctcggcccccagctggaacaccacggtcaggcttctccggcgctgccgtgtgctgtgcaatgggggctcctcctctcactccacaggggaggttgtggtgactatggagccagaggtacccatcaagaaactggagaccatggtgaagctggacgcgacttctgaagctgttgtcaaggtggatgtggctgaggaggagaaggagaagaagaagaagaagaagggcactgcggaggagccagaggaggaggagccagacgagagcatgctggactggtggtccaagtactttgcctccattgacaccatgaaggagcaacttcgacaacaagagccctctggaattgacttggaggagaaggaggaagtggacaataccgagggcctgaaggggtcaatgaagggcaaggagaaggcaagggctgccaaagaggagaagaagaagaaaactcagagctctggctctggccaggggtccgaggcccccgagaagaagaaacccaagattgatgagcttaaggtataccccaaagagctggagtccgagtttgataactttgaggactggctgcacactttcaacttgcttcggggcaagaccggggatgatgaggatggctccaccgaggaggagcgcattgtgggacgcttcaagggctccctctgcgtgtacaaagtgccactcccagaggacgtgtcccgggaagccggctacgactccacctacggcatgttccagggcatcccgagcaatgaccccatcaatgtgctggtccgagtctatgtggtccgggccacggacctgcaccctgctgacatcaacggcaaagctgacccctacatcgccatccggctaggcaagactgacatccgcgacaaggagaactacatctccaagcagctcaaccctgtctttgggaagtcctttgacatcgaggcctccttccccatggaatccatgctgacggtggctgtgtatgactgggacctggtgggcactgatgacctcattggggaaaccaagatcgacctggagaaccgcttctacagcaagcaccgcgccacctgcggcatcgcccagacctactccacacatggctacaatatctggcgggaccccatgaagcccagccagatcctgacccgcctctgcaaagacggcaaagtggacggcccccactttgggccccctgggagagtgaaggtggccaaccgcgtcttcactgggccctctgagattgaggacgagaacggtcagaggaagcccacagacgagcatgtggcgctgttggccctgaggcactgggaggacatcccccgcgcaggctgccgcctggtgccagagcatgtggagacgaggccgctgctcaaccccgacaagccgggcatcgagcagggccgcctggagctgtgggtggacatgttccccatggacatgccagcccctgggacgcctctggacatctcacctcggaagcccaagaagtacgagctgcgggtcatcatctggaacacagatgaggtggtcttggaggacgacgacttcttcacaggggagaagtccagtgacatcttcgtgagggggtggctgaagggccagcaggaggacaagcaggacacagacgtccactaccactccctcactggcgagggcaacttcaactggcgctacctgttccccttcgactacctggcggcggaggagaagatcgtcatctccaagaaggagtccatgttctcctgggacgagaccgagtacaagatccccgcgcggctcaccctgcagatctgggatgcggaccacttctccgctgacgacttcctgggggccatcgagctggacctgaaccggttcccgcggggcgcaaagacagccaagcagtgcaccatggagatggccaccggggaggtggacgtgcccctcgtgtccatcttcaagcaaaagcgcgtcaaaggctggtggcccctcctggcccgcaatgagaacgatgagtttgagctcacgggcaaggtggaggctgagctgcatttactgacagcagaggaggcagagaagaacccagtgggcctggcccgcaatgaacctgaccccctagagaaacccaaccggcccgacacggccttcgtctggttcctcaaccctctcaagtccatcaagtacctcatctgcacccggtacaagtggctcatcatcaagatcgtgctggcgctgttggggctgctcatgttggggctcttcctctacagcctccctggctacatggtcaaaaagctccttggggcatga

SEQ ID NO: 24 - protein, 1260 aa, homo sapiens
MMTDTQDGPSESSQIMRSLTPLINREEAFGEAGEAGLWPSITHTPDSQEEGLNDIQEMIKTEKSYPERRLRGVLEELSCGCCRFLSLADKDQGHSSRTRLDRERLKSCMRELENMGQQARMLRAQVKRHTVRDKLRLCQNFLQKLRFLADEPQHSIPDIFIWMMSNNKRVAYARVPSKDLLFSIVEEETGKDCAKVKTLFLKLPGKRGFGSAGWTVQAKVELYLWLGLSKQRKEFLCGLPCGFQEVKAAQGLGLHAFPPVSLVYTKKQAFQLRAHMYQARSLFAADSSGLSDPFARVFFINQSQCTEVLNETLCPTWDQMLVFDNLELYGEAHELRDDPPIIVIEIYDQDSMGKADFMGRTFAKPLVKMADEAYCPPRFPPQLEYYQIYRGNATAGDLLAAFELLQIGPAGKADLPPINGPVDVDRGPIMPVPMGIRPVLSKYRVEVLFWGLRDLKRVNLAQVDRPRVDIECAGKGVQSSLIHNYKKNPNFNTLVKWFEVDLPENELLHPPLNIRVVDCRAFGRYTLVGSHAVSSLRRFIYRPPDRSAPSWNTTVRLLRRCRVLCNGGSSSHSTGEVVVTMEPEVPIKKLETMVKLDATSEAVVKVDVAEEEKEKKKKKKGTAEEPEEEEPDESMLDWWSKYFASIDTMKEQLRQQEPSGIDLEEKEEVDNTEGLKGSMKGKEKARAAKEEKKKKTQSSGSGQGSEAPEKKKPKIDELKVYPKELESEFDNFEDWLHTFNLLRGKTGDDEDGSTEEERIVGRFKGSLCVYKVPLPEDVSREAGYDSTYGMFQGIPSNDPINVLVRVYVVRATDLHPADINGKADPYIAIRLGKTDIRDKENYISKQLNPVFGKSFDIEASFPMESMLTVAVYDWDLVGTDDLIGETKIDLENRFYSKHRATCGIAQTYSTHGYNIWRDPMKPSQILTRLCKDGKVDGPHFGPPGRVKVANRVFTGPSEIEDENGQRKPTDEHVALLALRHWEDIPRAGCRLVPEHVETRPLLNPDKPGIEQGRLELWVDMFPMDMPAPGTPLDISPRKPKKYELRVIIWNTDEVVLEDDDFFTGEKSSDIFVRGWLKGQQEDKQDTDVHYHSLTGEGNFNWRYLFPFDYLAAEEKIVISKKESMFSWDETEYKIPARLTLQIWDADHFSADDFLGAIELDLNRFPRGAKTAKQCTMEMATGEVDVPLVSIFKQKRVKGWWPLLARNENDEFELTGKVEAELHLLTAEEAEKNPVGLARNEPDPLEKPNRPDTSFIWFLNP